European Patent Specification EP 3 817 762 B1, published August 5, 2026. Title: MULTIFUNCTIONAL PROTEIN MOLECULES COMPRISING DECORIN AND USE THEREOF. Applicant: CATALENT PHARMA SOLUTIONS, LLC. Application EP 19830823.1. The sequence listing filed with the application follows.

SEQUENCE LISTING (67 sequences)

SEQ ID NO: 1 - DNA, 2424 bp, Artificial Sequence
  synthetic
atgatgtcctttgtctctctgctcctggttggcatcctattccatgccacccaggccgaggtgcagctggtggagtctgggggaggcttggtacagcctggggggtccctgagactctcctgtgcagcctctggatacacctttaccaactatggcatgaactgggtccgccaggctccagggaaggggctggagtgggtgggctggataaacacttacactggtgagccaacatatgcagctgacttcaagcgccggtttaccttctctttggacacctccaagtccacggcctatctgcaaatgaacagcctgcgggccgaggacacggccgtatattactgtgcgaaatacccccactactacggtagtagccactggtactttgacgtgtggggccagggaaccctggtcaccgtctcctcagcctccaccaagggcccatcggtcttccccctggcaccctcctccaagagcacctctgggggcacagcggccctgggctgcctggtcaaggactacttccccgaaccggtgacggtgtcgtggaactcaggcgccctgaccagcggcgtgcacaccttcccggctgtcctacagtcctcaggactctactccctcagcagcgtggtgaccgtgccctccagcagcttgggcacccagacctacatctgcaacgtgaatcacaagcccagcaacaccaaggtggacaagaaagttgagcccaaatcttgtgacaaaactcacacatgcccaccgtgcccagcacctgaactcctggggggaccgtcagtcttcctcttccccccaaaacccaaggacaccctcatgatctcccggacccctgaggtcacatgcgtggtggtggacgtgagccacgaagaccctgaggtcaagttcaactggtacgtggacggcgtggaggtgcataatgccaagacaaagccgcgggaggagcagtacaacagcacgtaccgggtggtcagcgtcctcaccgtcctgcaccaggactggctgaatggcaaggagtacaagtgcaaggtctccaacaaagccctcccagcccccatcgagaaaaccatctccaaagccaaagggcagccccgagaaccacaggtgtacaccctgcccccatcccgggaggagatgaccaagaaccaggtcagcctgacctgcctggtcaaaggcttctatcccagcgacatcgccgtggagtgggagagcaatgggcagccggagaacaactacaagaccacgcctcccgtgctggactccgacggctccttcttcctctacagcaagctcaccgtggacaagagcaggtggcagcaggggaacgtcttctcatgctccgtgatgcatgaggctctgcacaaccactacacgcagaagagcctctccctgtctcccgggaaatccgggggtggcggatccgatgaggctgcagggataggcccagaagttcctgatgaccgcgacttcgagccctccctaggcccagtgtgccccttccgctgtcaatgccatcttcgagtggtccagtgttctgatttgggtctggacaaagtgccaaaggatcttccccctgacacaactctgctagacctgcaaaacaacaaaataaccgaaatcaaagatggagactttaagaacctgaagaaccttcacgcattgattcttgtcaacaataaaattagcaaagttagtcctggagcatttacacctttggtgaagttggaacgactttatctgtccaagaatcagctgaaggaattgccagaaaaaatgcccaaaactcttcaggagctgcgtgcccatgagaatgagatcaccaaagtgcgaaaagttactttcaatggactgaaccagatgattgtcatagaactgggcaccaatccgctgaagagctcaggaattgaaaatggggctttccagggaatgaagaagctctcctacatccgcattgctgataccaatatcaccagcattcctcaaggtcttcctccttcccttacggaattacatcttgatggcaacaaaatcagcagagttgatgcagctagcctgaaaggactgaataatttggctaagttgggattgagtttcaacagcatctctgctgttgacaatggctctctggccaacacgcctcatctgagggagcttcacttggacaacaacaagcttaccagagtacctggtgggctggcagagcataagtacatccaggttgtctaccttcataacaacaatatctctgtagttggatcaagtgacttctgcccacctggacacaacaccaaaaaggcttcttattcgggtgtgagtcttttcagcaacccggtccagtactgggagatacagccatccaccttcagatgtgtctacgtgcgctctgccattcaactcggaaactataagtga

SEQ ID NO: 2 - protein, 807 aa, Artificial Sequence
  synthetic
MMSFVSLLLVGILFHATQAEVQLVESGGGLVQPGGSLRLSCAASGYTFTNYGMNWVRQAPGKGLEWVGWINTYTGEPTYAADFKRRFTFSLDTSKSTAYLQMNSLRAEDTAVYYCAKYPHYYGSSHWYFDVWGQGTLVTVSSASTKGPSVFPLAPSSKSTSGGTAALGCLVKDYFPEPVTVSWNSGALTSGVHTFPAVLQSSGLYSLSSVVTVPSSSLGTQTYICNVNHKPSNTKVDKKVEPKSCDKTHTCPPCPAPELLGGPSVFLFPPKPKDTLMISRTPEVTCVVVDVSHEDPEVKFNWYVDGVEVHNAKTKPREEQYNSTYRVVSVLTVLHQDWLNGKEYKCKVSNKALPAPIEKTISKAKGQPREPQVYTLPPSREEMTKNQVSLTCLVKGFYPSDIAVEWESNGQPENNYKTTPPVLDSDGSFFLYSKLTVDKSRWQQGNVFSCSVMHEALHNHYTQKSLSLSPGKSGGGGSDEAAGIGPEVPDDRDFEPSLGPVCPFRCQCHLRVVQCSDLGLDKVPKDLPPDTTLLDLQNNKITEIKDGDFKNLKNLHALILVNNKISKVSPGAFTPLVKLERLYLSKNQLKELPEKMPKTLQELRAHENEITKVRKVTFNGLNQMIVIELGTNPLKSSGIENGAFQGMKKLSYIRIADTNITSIPQGLPPSLTELHLDGNKISRVDAASLKGLNNLAKLGLSFNSISAVDNGSLANTPHLRELHLDNNKLTRVPGGLAEHKYIQVVYLHNNNISVVGSSDFCPPGHNTKKASYSGVSLFSNPVQYWEIQPSTFRCVYVRSAIQLGNYK

SEQ ID NO: 3 - DNA, 702 bp, Artificial Sequence
  synthetic
atgatgtcctttgtctctctgctcctggttggcatcctgttccatgccacccaggccgacatccagatgacccagtctccatcctccctgtctgcatctgtaggagacagagtcaccatcacttgcagtgcaagtcaggacattagcaattatttaaactggtatcagcagaaaccagggaaagctcctaaggtcctgatctatttcacatccagtttgcactcaggggtcccatctaggttcagtggcagtggatctgggacagatttcactctcaccatcagcagcctgcagcctgaagattttgcaacttattactgccaacagtatagtaccgtgccttggacgttcggccaagggaccaaggtggaaatcaaacgaactgtggctgcaccatctgtcttcatcttcccgccatctgatgagcagcttaagtccggaactgctagcgttgtgtgcctgctgaataacttctatcccagagaggccaaagtacagtggaaggtggataacgccctccaatcgggtaactcccaggagagtgtcacagagcaggacagcaaggacagcacctacagcctcagcagcaccctgacgctgagcaaagcagactacgagaaacacaaagtctacgcctgcgaagtcacccatcagggcctgagctcgcccgtcacaaagagcttcaacaggggagagtgttag

SEQ ID NO: 4 - protein, 233 aa, Artificial Sequence
  synthetic
MMSFVSLLLVGILFHATQADIQMTQSPSSLSASVGDRVTITCSASQDISNYLNWYQQKPGKAPKVLIYFTSSLHSGVPSRFSGSGSGTDFTLTISSLQPEDFATYYCQQYSTVPWTFGQGTKVEIKRTVAAPSVFIFPPSDEQLKSGTASVVCLLNNFYPREAKVQWKVDNALQSGNSQESVTEQDSKDSTYSLSSTLTLSKADYEKHKVYACEVTHQGLSSPVTKSFNRGEC

SEQ ID NO: 5 - protein, 19 aa, Artificial Sequence
  synthetic
MMSFVSLLLVGILFHATQA

SEQ ID NO: 6 - protein, 6 aa, Artificial Sequence
  synthetic
SGGGGS

SEQ ID NO: 7 - protein, 329 aa, Artificial Sequence
  synthetic
DEAAGIGPEVPDDRDFEPSLGPVCPFRCQCHLRVVQCSDLGLDKVPKDLPPDTTLLDLQNNKITEIKDGDFKNLKNLHALILVNNKISKVSPGAFTPLVKLERLYLSKNQLKELPEKMPKTLQELRAHENEITKVRKVTFNGLNQMIVIELGTNPLKSSGIENGAFQGMKKLSYIRIADTNITSIPQGLPPSLTELHLDGNKISRVDAASLKGLNNLAKLGLSFNSISAVDNGSLANTPHLRELHLDNNKLTRVPGGLAEHKYIQVVYLHNNNISVVGSSDFCPPGHNTKKASYSGVSLFSNPVQYWEIQPSTFRCVYVRSAIQLGNYK

SEQ ID NO: 8 - protein, 453 aa, Artificial Sequence
  synthetic
EVQLVESGGGLVQPGGSLRLSCAASGYTFTNYGMNWVRQAPGKGLEWVGWINTYTGEPTYAADFKRRFTFSLDTSKSTAYLQMNSLRAEDTAVYYCAKYPHYYGSSHWYFDVWGQGTLVTVSSASTKGPSVFPLAPSSKSTSGGTAALGCLVKDYFPEPVTVSWNSGALTSGVHTFPAVLQSSGLYSLSSVVTVPSSSLGTQTYICNVNHKPSNTKVDKKVEPKSCDKTHTCPPCPAPELLGGPSVFLFPPKPKDTLMISRTPEVTCVVVDVSHEDPEVKFNWYVDGVEVHNAKTKPREEQYNSTYRVVSVLTVLHQDWLNGKEYKCKVSNKALPAPIEKTISKAKGQPREPQVYTLPPSREEMTKNQVSLTCLVKGFYPSDIAVEWESNGQPENNYKTTPPVLDSDGSFFLYSKLTVDKSRWQQGNVFSCSVMHEALHNHYTQKSLSLSPGK

SEQ ID NO: 9 - protein, 214 aa, Artificial Sequence
  synthetic
DIQMTQSPSSLSASVGDRVTITCSASQDISNYLNWYQQKPGKAPKVLIYFTSSLHSGVPSRFSGSGSGTDFTLTISSLQPEDFATYYCQQYSTVPWTFGQGTKVEIKRTVAAPSVFIFPPSDEQLKSGTASVVCLLNNFYPREAKVQWKVDNALQSGNSQESVTEQDSKDSTYSLSSTLTLSKADYEKHKVYACEVTHQGLSSPVTKSFNRGEC

SEQ ID NO: 10 - DNA, 2409 bp, Artificial Sequence
  synthetic
atgatgtcctttgtctctctgctcctggttggcatcctattccatgccacccaggcccaggtgcagctggtggagtccggcggcggcgtcgtgcagcccggccggtccctgcggctgtcctgcgccgcctccggcttcaccttctcctcctacaccatgcactgggtgcggcaggcccccggcaagggcctggagtgggtgactttcatctcctacgacggcaacaacaagtactacgccgactccgtgaagggccggttcaccatctcccgcgacaactccaagaacaccctgtacctgcagatgaactccctgcgggccgaggacaccgccatctactactgcgcccggaccggctggctgggccccttcgactactggggccagggcaccctggtgaccgtgtcctccgcctccaccaagggcccatcggtcttccccctggcaccctctagcaagagcacctctgggggcacagcggccctgggctgcctggtcaaggactacttccccgaaccggtgacggtgtcgtggaactcaggcgccctgaccagcggcgtgcacaccttcccggctgtcctacagtcctcaggactctactccctcagcagcgtggtgaccgtgccctccagcagcttgggcacccagacctacatctgcaacgtgaatcacaagcccagcaacaccaaggtggacaagcgggttgagcccaaatcttgtgacaaaactcacacatgcccaccgtgcccagcacctgaactcctggggggaccgtcagtcttcctcttccccccaaaacccaaggacaccctcatgatctcccggacccctgaggtcacatgcgtggtggtggacgtgagccacgaagaccctgaggtcaagttcaactggtacgtggacggcgtggaggtgcataatgccaagacaaagccgcgggaggagcagtacaacagcacgtaccgtgtggtcagcgtcctcaccgtcctgcaccaggactggctgaatggcaaggagtacaagtgcaaggtctccaacaaagccctcccagcccccatcgagaaaaccatctccaaagccaaagggcagccccgagaaccacaggtgtacaccctgcctccatcccgcgatgagctgaccaagaaccaggtcagcctgacctgcctggtcaaaggcttctatcccagcgacatcgccgtggagtgggagagcaatgggcagccggagaacaactacaagaccacgcctcccgtgctggactccgacggctccttcttcctctatagcaagctcaccgtggacaagagcaggtggcagcaggggaacgtcttctcatgctccgtgatgcatgaggctctgcacaaccactacacgcagaagagcctctccctgtctcctgggaaatccgggggtggcggatccgatgaggctgcagggataggcccagaagttcctgatgaccgcgacttcgagccctccctaggcccagtgtgccccttccgctgtcaatgccatcttcgagtggtccagtgttctgatttgggtctggacaaagtgccaaaggatcttccccctgacacaactctgctagacctgcaaaacaacaaaataaccgaaatcaaagatggagactttaagaacctgaagaaccttcacgcattgattcttgtcaacaataaaattagcaaagttagtcctggagcatttacacctttggtgaagttggaacgactttatctgtccaagaatcagctgaaggaattgccagaaaaaatgcccaaaactcttcaggagctgcgtgcccatgagaatgagatcaccaaagtgcgaaaagttactttcaatggactgaaccagatgattgtcatagaactgggcaccaatccgctgaagagctcaggaattgaaaatggggctttccagggaatgaagaagctctcctacatccgcattgctgataccaatatcaccagcattcctcaaggtcttcctccttcccttacggaattacatcttgatggcaacaaaatcagcagagttgatgcagctagcctgaaaggactgaataatttggctaagttgggattgagtttcaacagcatctctgctgttgacaatggctctctggccaacacgcctcatctgagggagcttcacttggacaacaacaagcttaccagagtacctggtgggctggcagagcataagtacatccaggttgtctaccttcataacaacaatatctctgtagttggatcaagtgacttctgcccacctggacacaacaccaaaaaggcttcttattcgggtgtgagtcttttcagcaacccggtccagtactgggagatacagccatccaccttcagatgtgtctacgtgcgctctgccattcaactcggaaactataagtga

SEQ ID NO: 11 - protein, 802 aa, Artificial Sequence
  synthetic
MMSFVSLLLVGILFHATQAQVQLVESGGGVVQPGRSLRLSCAASGFTFSSYTMHWVRQAPGKGLEWVTFISYDGNNKYYADSVKGRFTISRDNSKNTLYLQMNSLRAEDTAIYYCARTGWLGPFDYWGQGTLVTVSSASTKGPSVFPLAPSSKSTSGGTAALGCLVKDYFPEPVTVSWNSGALTSGVHTFPAVLQSSGLYSLSSVVTVPSSSLGTQTYICNVNHKPSNTKVDKRVEPKSCDKTHTCPPCPAPELLGGPSVFLFPPKPKDTLMISRTPEVTCVVVDVSHEDPEVKFNWYVDGVEVHNAKTKPREEQYNSTYRVVSVLTVLHQDWLNGKEYKCKVSNKALPAPIEKTISKAKGQPREPQVYTLPPSRDELTKNQVSLTCLVKGFYPSDIAVEWESNGQPENNYKTTPPVLDSDGSFFLYSKLTVDKSRWQQGNVFSCSVMHEALHNHYTQKSLSLSPGKSGGGGSDEAAGIGPEVPDDRDFEPSLGPVCPFRCQCHLRVVQCSDLGLDKVPKDLPPDTTLLDLQNNKITEIKDGDFKNLKNLHALILVNNKISKVSPGAFTPLVKLERLYLSKNQLKELPEKMPKTLQELRAHENEITKVRKVTFNGLNQMIVIELGTNPLKSSGIENGAFQGMKKLSYIRIADTNITSIPQGLPPSLTELHLDGNKISRVDAASLKGLNNLAKLGLSFNSISAVDNGSLANTPHLRELHLDNNKLTRVPGGLAEHKYIQVVYLHNNNISVVGSSDFCPPGHNTKKASYSGVSLFSNPVQYWEIQPSTFRCVYVRSAIQLGNYK

SEQ ID NO: 12 - DNA, 705 bp, Artificial Sequence
  synthetic
atgatgtcctttgtctctctgctcctggttggcatcctattccatgccacccaggccgagatcgtgctgacccagtcccccggcaccctgtccctgtcccccggcgagcgggccaccctgtcctgccgggcctcccagtccgtgggctcctcctacctggcctggtaccagcagaagcccggccaggccccccggctgctgatctacggcgccttctcccgcgccaccggcatccccgaccggttctccggctccggctccggcaccgacttcaccctgaccatctcccggctggagcccgaggacttcgccgtgtactactgccagcagtacggctcctccccctggaccttcggccagggcaccaaggtggagatcaagcgaactgtggctgcaccatctgtcttcatcttcccgccatctgatgagcagcttaagtccggaactgctagcgttgtgtgcctgctgaataacttctatcccagagaggccaaagtacagtggaaggtggataacgccctccaatcgggtaactcccaggagagtgtcacagagcaggacagcaaggacagcacctacagcctcagcagcaccctgacgctgagcaaagcagactacgagaaacacaaagtctacgcctgcgaagtcacccatcagggcctgagctcgcccgtcacaaagagcttcaacaggggagagtgttag

SEQ ID NO: 13 - protein, 234 aa, Artificial Sequence
  synthetic
MMSFVSLLLVGILFHATQAEIVLTQSPGTLSLSPGERATLSCRASQSVGSSYLAWYQQKPGQAPRLLIYGAFSRATGIPDRFSGSGSGTDFTLTISRLEPEDFAVYYCQQYGSSPWTFGQGTKVEIKRTVAAPSVFIFPPSDEQLKSGTASVVCLLNNFYPREAKVQWKVDNALQSGNSQESVTEQDSKDSTYSLSSTLTLSKADYEKHKVYACEVTHQGLSSPVTKSFNRGEC

SEQ ID NO: 14 - protein, 448 aa, Artificial Sequence
  synthetic
QVQLVESGGGVVQPGRSLRLSCAASGFTFSSYTMHWVRQAPGKGLEWVTFISYDGNNKYYADSVKGRFTISRDNSKNTLYLQMNSLRAEDTAIYYCARTGWLGPFDYWGQGTLVTVSSASTKGPSVFPLAPSSKSTSGGTAALGCLVKDYFPEPVTVSWNSGALTSGVHTFPAVLQSSGLYSLSSVVTVPSSSLGTQTYICNVNHKPSNTKVDKRVEPKSCDKTHTCPPCPAPELLGGPSVFLFPPKPKDTLMISRTPEVTCVVVDVSHEDPEVKFNWYVDGVEVHNAKTKPREEQYNSTYRVVSVLTVLHQDWLNGKEYKCKVSNKALPAPIEKTISKAKGQPREPQVYTLPPSRDELTKNQVSLTCLVKGFYPSDIAVEWESNGQPENNYKTTPPVLDSDGSFFLYSKLTVDKSRWQQGNVFSCSVMHEALHNHYTQKSLSLSPGK

SEQ ID NO: 15 - protein, 215 aa, Artificial Sequence
  synthetic
EIVLTQSPGTLSLSPGERATLSCRASQSVGSSYLAWYQQKPGQAPRLLIYGAFSRATGIPDRFSGSGSGTDFTLTISRLEPEDFAVYYCQQYGSSPWTFGQGTKVEIKRTVAAPSVFIFPPSDEQLKSGTASVVCLLNNFYPREAKVQWKVDNALQSGNSQESVTEQDSKDSTYSLSSTLTLSKADYEKHKVYACEVTHQGLSSPVTKSFNRGEC

SEQ ID NO: 16 - DNA, 2409 bp, Artificial Sequence
  synthetic
atgatgtcctttgtctctctgctcctggttggcatcctattccatgccacccaggccgaggtacaactcgtggaatccggcgggggactcgtccaaccgggtggtagtctcaggttgagctgcgctgcgagcggtttcactttctcagactcatggattcattgggtgcgccaagcacctggaaaagggttggaatgggttgcctggatctctccttacggaggttctacctactacgctgattcagtaaaggggcggttcacaatttcagccgatacttccaaaaatacggcttacctgcaaatgaactctttgagggcggaggatacggcggtctactactgtgcacgcaggcactggcctggagggttcgattattggggtcaaggcactttggtaaccgtatcctccgcttctaccaaaggcccatcagtatttcctttggctcccagctctaagtccacttccggtggaactgccgcacttggatgtctcgtcaaagactactttcctgagccggtaactgtgtcatggaactccggcgccctcactagcggcgtccatacatttccagcggttctccagtcaagtggcctctacagcctgtccagtgtagttactgtcccgtcttctagtctgggaacgcaaacatatatttgcaatgtgaatcataagcctagtaacacaaaagtcgataaaaaagtggagccgaaaagttgtgacaaaacgcatacctgtccgccttgtccggcccccgaactcttgggcggcccatcagtctttctcttcccgcccaaacctaaggacacgttgatgataagtcgcacgcccgaggttacatgcgtcgtagtcgatgtcagccacgaggatccggaggtaaagtttaactggtatgtagacggagttgaagtacacaacgccaaaactaaaccgagagaggagcagtacgcatcaacctatcgcgtagtatctgtattgacggtccttcaccaagactggctcaatgggaaagaatacaagtgcaaagtttctaataaagccctccctgcaccaatcgaaaagactatttcaaaagccaaaggacaaccaagagaaccacaagtttatacattgccacctagtcgcgaggagatgactaaaaaccaagtgtcccttacttgtctcgtaaagggtttctatccaagcgacatagcagttgagtgggaaagtaatggccagccggaaaacaactacaagacgacccccccggttctcgactccgatggatcattctttttgtatagtaaactcacagttgataagagtcgatggcagcaggggaatgttttttcttgctctgtgatgcacgaggcgctccacaaccactatacgcaaaagtccctcagcctgagccccgggaaatccgggggtggcggatccgatgaggctgcagggataggcccagaagttcctgatgaccgcgacttcgagccctccctaggcccagtgtgccccttccgctgtcaatgccatcttcgagtggtccagtgttctgatttgggtctggacaaagtgccaaaggatcttccccctgacacaactctgctagacctgcaaaacaacaaaataaccgaaatcaaagatggagactttaagaacctgaagaaccttcacgcattgattcttgtcaacaataaaattagcaaagttagtcctggagcatttacacctttggtgaagttggaacgactttatctgtccaagaatcagctgaaggaattgccagaaaaaatgcccaaaactcttcaggagctgcgtgcccatgagaatgagatcaccaaagtgcgaaaagttactttcaatggactgaaccagatgattgtcatagaactgggcaccaatccgctgaagagctcaggaattgaaaatggggctttccagggaatgaagaagctctcctacatccgcattgctgataccaatatcaccagcattcctcaaggtcttcctccttcccttacggaattacatcttgatggcaacaaaatcagcagagttgatgcagctagcctgaaaggactgaataatttggctaagttgggattgagtttcaacagcatctctgctgttgacaatggctctctggccaacacgcctcatctgagggagcttcacttggacaacaacaagcttaccagagtacctggtgggctggcagagcataagtacatccaggttgtctaccttcataacaacaatatctctgtagttggatcaagtgacttctgcccacctggacacaacaccaaaaaggcttcttattcgggtgtgagtcttttcagcaacccggtccagtactgggagatacagccatccaccttcagatgtgtctacgtgcgctctgccattcaactcggaaactataagtga

SEQ ID NO: 17 - protein, 802 aa, Artificial Sequence
  synthetic
MMSFVSLLLVGILFHATQAEVQLVESGGGLVQPGGSLRLSCAASGFTFSDSWIHWVRQAPGKGLEWVAWISPYGGSTYYADSVKGRFTISADTSKNTAYLQMNSLRAEDTAVYYCARRHWPGGFDYWGQGTLVTVSSASTKGPSVFPLAPSSKSTSGGTAALGCLVKDYFPEPVTVSWNSGALTSGVHTFPAVLQSSGLYSLSSVVTVPSSSLGTQTYICNVNHKPSNTKVDKKVEPKSCDKTHTCPPCPAPELLGGPSVFLFPPKPKDTLMISRTPEVTCVVVDVSHEDPEVKFNWYVDGVEVHNAKTKPREEQYASTYRVVSVLTVLHQDWLNGKEYKCKVSNKALPAPIEKTISKAKGQPREPQVYTLPPSREEMTKNQVSLTCLVKGFYPSDIAVEWESNGQPENNYKTTPPVLDSDGSFFLYSKLTVDKSRWQQGNVFSCSVMHEALHNHYTQKSLSLSPGKSGGGGSDEAAGIGPEVPDDRDFEPSLGPVCPFRCQCHLRVVQCSDLGLDKVPKDLPPDTTLLDLQNNKITEIKDGDFKNLKNLHALILVNNKISKVSPGAFTPLVKLERLYLSKNQLKELPEKMPKTLQELRAHENEITKVRKVTFNGLNQMIVIELGTNPLKSSGIENGAFQGMKKLSYIRIADTNITSIPQGLPPSLTELHLDGNKISRVDAASLKGLNNLAKLGLSFNSISAVDNGSLANTPHLRELHLDNNKLTRVPGGLAEHKYIQVVYLHNNNISVVGSSDFCPPGHNTKKASYSGVSLFSNPVQYWEIQPSTFRCVYVRSAIQLGNYK

SEQ ID NO: 18 - DNA, 702 bp, Artificial Sequence
  synthetic
atgatgtcctttgtctctctgctcctggttggcatcctattccatgccacccaggccgacattcagatgacacaatcacctagcagtctgagtgcgagcgtaggtgatcgcgtaacgattacctgcagggcctctcaagacgtgtcaacggcagtggcgtggtaccagcagaagcctggtaaagctcctaagctcctcatctattcagcttccttcttgtatagtggagtaccgtcaagattttccggaagcggatcaggtacagattttactttgactatcagtagtttgcagccagaggatttcgctacatattactgtcaacaatatctctatcaccctgccacttttggacaagggactaaagtcgaaataaaacgaacagtggccgcaccaagcgtttttatctttcccccatccgacgagcagttgaagagcggcaccgcgtccgtggtctgcctgttgaataatttctatccaagggaggcaaaagtgcaatggaaagttgataatgcgcttcaatccggaaactcacaagaatcagtaacagaacaagactctaaagacagtacatattctcttagtagcacactcactctttcaaaggctgactatgagaaacataaagtgtacgcttgtgaagtgacacatcaaggtcttagctccccagtaactaagagctttaataggggcgagtgctga

SEQ ID NO: 19 - protein, 233 aa, Artificial Sequence
  synthetic
MMSFVSLLLVGILFHATQADIQMTQSPSSLSASVGDRVTITCRASQDVSTAVAWYQQKPGKAPKLLIYSASFLYSGVPSRFSGSGSGTDFTLTISSLQPEDFATYYCQQYLYHPATFGQGTKVEIKRTVAAPSVFIFPPSDEQLKSGTASVVCLLNNFYPREAKVQWKVDNALQSGNSQESVTEQDSKDSTYSLSSTLTLSKADYEKHKVYACEVTHQGLSSPVTKSFNRGEC

SEQ ID NO: 20 - protein, 448 aa, Artificial Sequence
  synthetic
EVQLVESGGGLVQPGGSLRLSCAASGFTFSDSWIHWVRQAPGKGLEWVAWISPYGGSTYYADSVKGRFTISADTSKNTAYLQMNSLRAEDTAVYYCARRHWPGGFDYWGQGTLVTVSSASTKGPSVFPLAPSSKSTSGGTAALGCLVKDYFPEPVTVSWNSGALTSGVHTFPAVLQSSGLYSLSSVVTVPSSSLGTQTYICNVNHKPSNTKVDKKVEPKSCDKTHTCPPCPAPELLGGPSVFLFPPKPKDTLMISRTPEVTCVVVDVSHEDPEVKFNWYVDGVEVHNAKTKPREEQYASTYRVVSVLTVLHQDWLNGKEYKCKVSNKALPAPIEKTISKAKGQPREPQVYTLPPSREEMTKNQVSLTCLVKGFYPSDIAVEWESNGQPENNYKTTPPVLDSDGSFFLYSKLTVDKSRWQQGNVFSCSVMHEALHNHYTQKSLSLSPGK

SEQ ID NO: 21 - protein, 214 aa, Artificial Sequence
  synthetic
DIQMTQSPSSLSASVGDRVTITCRASQDVSTAVAWYQQKPGKAPKLLIYSASFLYSGVPSRFSGSGSGTDFTLTISSLQPEDFATYYCQQYLYHPATFGQGTKVEIKRTVAAPSVFIFPPSDEQLKSGTASVVCLLNNFYPREAKVQWKVDNALQSGNSQESVTEQDSKDSTYSLSSTLTLSKADYEKHKVYACEVTHQGLSSPVTKSFNRGEC

SEQ ID NO: 22 - DNA, 2415 bp, Artificial Sequence
  synthetic
atgatgtcctttgtctctctgctcctggttggcatcctattccatgccacccaggccgaggtacagcttttggagtcaggcggggggctcgtccaacctggggggtcactccggttgtcatgtgctgccagtggcttcacattctcatcttacattatgatgtgggttcgacaggcccctgggaaggggctggagtgggtttcctccatctacccctccgggggaattaccttctatgccgacacggtaaagggtcgcttcactataagtcgagataacagcaaaaatacgctgtatctccagatgaactctctcagggctgaggacacagctgtatattactgcgcgcggattaagttggggaccgtcacaacagtggattactggggtcaaggcactctggtaaccgtatcctcagcatccaccaagggcccaagtgtattcccgctggccccttcaagtaaatccacgtctggcggcacagccgctctcggttgcctggttaaggactacttcccagaacctgtcactgtcagttggaactcaggcgcattgacatctggtgtccatacattccccgcagtcctgcaaagctctggactttacagtcttagtagcgtagtgacagtcccatcttcaagtcttgggacccaaacttatatttgcaacgtaaatcataaaccctccaacactaaagtagacaaaaaagtagagccgaaatcttgcgacaaaacgcatacatgcccaccatgtcccgctccggaactcctgggcggcccgtccgtttttctctttcccccaaagcccaaggatacgcttatgatcagcagaacaccggaagttacttgtgtagtcgttgacgtgtctcacgaagatcccgaagtcaaatttaattggtatgtggatggcgtcgaagtgcacaacgcaaaaaccaaacccagagaggaacagtataacagcacgtatcgagtggtctccgtacttacggtcctccaccaggactggttgaatggcaaggagtacaagtgcaaagtgagcaataaagcgttgccagccccgatcgaaaaaaccatcagcaaggccaagggacagcctagagagccgcaggtttacaccttgccgccatcaagggatgaactgactaaaaaccaggtatccctgacctgcctggttaagggtttttaccccagtgatatagcggttgaatgggagtctaacgggcagccagagaacaactacaaaacgacacctcccgttctggattccgatggcagctttttcttgtattctaaactcaccgtggataaatcccgatggcagcaaggcaacgtcttctcctgcagcgtgatgcatgaagccttgcacaaccactatacccaaaagagtctcagcctgtcacccgggaaatccgggggtggcggatccgatgaggctgcagggataggcccagaagttcctgatgaccgcgacttcgagccctccctaggcccagtgtgccccttccgctgtcaatgccatcttcgagtggtccagtgttctgatttgggtctggacaaagtgccaaaggatcttccccctgacacaactctgctagacctgcaaaacaacaaaataaccgaaatcaaagatggagactttaagaacctgaagaaccttcacgcattgattcttgtcaacaataaaattagcaaagttagtcctggagcatttacacctttggtgaagttggaacgactttatctgtccaagaatcagctgaaggaattgccagaaaaaatgcccaaaactcttcaggagctgcgtgcccatgagaatgagatcaccaaagtgcgaaaagttactttcaatggactgaaccagatgattgtcatagaactgggcaccaatccgctgaagagctcaggaattgaaaatggggctttccagggaatgaagaagctctcctacatccgcattgctgataccaatatcaccagcattcctcaaggtcttcctccttcccttacggaattacatcttgatggcaacaaaatcagcagagttgatgcagctagcctgaaaggactgaataatttggctaagttgggattgagtttcaacagcatctctgctgttgacaatggctctctggccaacacgcctcatctgagggagcttcacttggacaacaacaagcttaccagagtacctggtgggctggcagagcataagtacatccaggttgtctaccttcataacaacaatatctctgtagttggatcaagtgacttctgcccacctggacacaacaccaaaaaggcttcttattcgggtgtgagtcttttcagcaacccggtccagtactgggagatacagccatccaccttcagatgtgtctacgtgcgctctgccattcaactcggaaactataagtga

SEQ ID NO: 23 - protein, 804 aa, Artificial Sequence
  synthetic
MMSFVSLLLVGILFHATQAEVQLLESGGGLVQPGGSLRLSCAASGFTFSSYIMMWVRQAPGKGLEWVSSIYPSGGITFYADTVKGRFTISRDNSKNTLYLQMNSLRAEDTAVYYCARIKLGTVTTVDYWGQGTLVTVSSASTKGPSVFPLAPSSKSTSGGTAALGCLVKDYFPEPVTVSWNSGALTSGVHTFPAVLQSSGLYSLSSVVTVPSSSLGTQTYICNVNHKPSNTKVDKKVEPKSCDKTHTCPPCPAPELLGGPSVFLFPPKPKDTLMISRTPEVTCVVVDVSHEDPEVKFNWYVDGVEVHNAKTKPREEQYNSTYRVVSVLTVLHQDWLNGKEYKCKVSNKALPAPIEKTISKAKGQPREPQVYTLPPSRDELTKNQVSLTCLVKGFYPSDIAVEWESNGQPENNYKTTPPVLDSDGSFFLYSKLTVDKSRWQQGNVFSCSVMHEALHNHYTQKSLSLSPGKSGGGGSDEAAGIGPEVPDDRDFEPSLGPVCPFRCQCHLRVVQCSDLGLDKVPKDLPPDTTLLDLQNNKITEIKDGDFKNLKNLHALILVNNKISKVSPGAFTPLVKLERLYLSKNQLKELPEKMPKTLQELRAHENEITKVRKVTFNGLNQMIVIELGTNPLKSSGIENGAFQGMKKLSYIRIADTNITSIPQGLPPSLTELHLDGNKISRVDAASLKGLNNLAKLGLSFNSISAVDNGSLANTPHLRELHLDNNKLTRVPGGLAEHKYIQVVYLHNNNISVVGSSDFCPPGHNTKKASYSGVSLFSNPVQYWEIQPSTFRCVYVRSAIQLGNYK

SEQ ID NO: 24 - DNA, 708 bp, Artificial Sequence
  synthetic
atgatgtcctttgtctctctgctcctggttggcatcctattccatgccacccaggcccagtctgcacttacacaaccggcgtccgtttccggatctccaggacagagcattactatcagttgcacgggaacctcctcagacgtaggggggtataattatgtgtcttggtatcaacagcatcccgggaaagcccccaaactgatgatctacgatgtcagcaatagaccaagcggtgtgagtaatcgatttagcgggtctaaatctggtaacacagcatccctcactattagtggactgcaagcagaagatgaggcagactattattgcagtagctatacgtctagttccacccgcgtttttggcactgggacgaaagtcaccgttctcggacaaccaaaagcaaaccccaccgtgactctgtttccgcctagcagcgaagaattgcaggccaataaggcgacactcgtatgccttatctccgacttctacccgggcgctgtgacagtcgcgtggaaagccgacggcagccctgttaaagctggagtcgagaccacgaagccgtccaagcagagtaacaataagtatgctgcatccagttatctctctctcactccggaacagtggaagtcccatcggtcctatagttgccaagtgacccatgagggttccaccgtagagaaaacggtagcacctaccgaatgtagttga

SEQ ID NO: 25 - protein, 235 aa, Artificial Sequence
  synthetic
MMSFVSLLLVGILFHATQAQSALTQPASVSGSPGQSITISCTGTSSDVGGYNYVSWYQQHPGKAPKLMIYDVSNRPSGVSNRFSGSKSGNTASLTISGLQAEDEADYYCSSYTSSSTRVFGTGTKVTVLGQPKANPTVTLFPPSSEELQANKATLVCLISDFYPGAVTVAWKADGSPVKAGVETTKPSKQSNNKYAASSYLSLTPEQWKSHRSYSCQVTHEGSTVEKTVAPTECS

SEQ ID NO: 26 - protein, 450 aa, Artificial Sequence
  synthetic
EVQLLESGGGLVQPGGSLRLSCAASGFTFSSYIMMWVRQAPGKGLEWVSSIYPSGGITFYADTVKGRFTISRDNSKNTLYLQMNSLRAEDTAVYYCARIKLGTVTTVDYWGQGTLVTVSSASTKGPSVFPLAPSSKSTSGGTAALGCLVKDYFPEPVTVSWNSGALTSGVHTFPAVLQSSGLYSLSSVVTVPSSSLGTQTYICNVNHKPSNTKVDKKVEPKSCDKTHTCPPCPAPELLGGPSVFLFPPKPKDTLMISRTPEVTCVVVDVSHEDPEVKFNWYVDGVEVHNAKTKPREEQYNSTYRVVSVLTVLHQDWLNGKEYKCKVSNKALPAPIEKTISKAKGQPREPQVYTLPPSRDELTKNQVSLTCLVKGFYPSDIAVEWESNGQPENNYKTTPPVLDSDGSFFLYSKLTVDKSRWQQGNVFSCSVMHEALHNHYTQKSLSLSPGK

SEQ ID NO: 27 - protein, 216 aa, Artificial Sequence
  synthetic
QSALTQPASVSGSPGQSITISCTGTSSDVGGYNYVSWYQQHPGKAPKLMIYDVSNRPSGVSNRFSGSKSGNTASLTISGLQAEDEADYYCSSYTSSSTRVFGTGTKVTVLGQPKANPTVTLFPPSSEELQANKATLVCLISDFYPGAVTVAWKADGSPVKAGVETTKPSKQSNNKYAASSYLSLTPEQWKSHRSYSCQVTHEGSTVEKTVAPTECS

SEQ ID NO: 28 - DNA, 2418 bp, Artificial Sequence
  synthetic
atgatgtcctttgtctctctgctcctggttggcatcctattccatgccacccaggccgaggtccagcttgttgaaagcggtggtggcctcgtgcagcctggtggcagtttgcggttgtcttgcgcagctagtggttttaccttctccagatactggatgtcatgggtccgacaggcccctggcaaggggcttgaatgggttgcaaatataaagcaggacggttctgaaaagtactatgtagactccgtcaaaggaagatttactattagtcgagacaacgccaagaatagcctctaccttcagatgaattctttgcgagcggaggacacagccgtatattactgcgcacgagaaggggggtggttcggtgaactggcttttgactactgggggcaaggtacgcttgtcacggtgagctctgcctctacaaaggggccgtctgtgtttccacttgctccatctagtaagtcaacttctggaggtactgcggcattgggatgccttgttaaggattattttcccgaacctgtaactgtgagctggaattcaggtgccctcacctctggtgtacatacctttccagcagttttgcaatcttccggtttgtactctcttagttcagttgtaactgtcccctcttcctctcttggtacccaaacatacatttgtaatgtcaatcacaaaccaagcaataccaaggtagacaagcgggtggaacccaaatcttgtgacaaaactcatacctgcccaccatgtcccgccccggagtttgaaggaggtccaagtgtatttcttttcccgcctaagcctaaggataccctcatgataagtcggacaccagaggtgacgtgtgttgtggtagacgtgagtcacgaagatcccgaagttaaatttaattggtatgtggacggggtggaagtccataacgcgaagacaaagccacgcgaagagcagtacaattccacgtacagggtggttagcgtgcttaccgtcctgcatcaagattggctgaacgggaaagaatacaaatgcaaagtatccaacaaggcgttgcctgcgagtatcgagaaaacgatttctaaagctaaaggacaaccccgggaaccccaggtctatacactgccgcccagcagagaagagatgacgaaaaatcaagtatcccttacgtgtctcgtcaaaggcttctacccttccgatattgctgtagagtgggaatctaacgggcagccggaaaataactacaagactactccgccagtacttgattcagacggctccttcttcctttattcaaaactcaccgtagataaaagtaggtggcaacaaggtaatgtttttagctgtagcgtaatgcacgaagcgttgcataaccattatacacagaaatcactcagcctgtcccccgggaaatccgggggtggcggatccgatgaggctgcagggataggcccagaagttcctgatgaccgcgacttcgagccctccctaggcccagtgtgccccttccgctgtcaatgccatcttcgagtggtccagtgttctgatttgggtctggacaaagtgccaaaggatcttccccctgacacaactctgctagacctgcaaaacaacaaaataaccgaaatcaaagatggagactttaagaacctgaagaaccttcacgcattgattcttgtcaacaataaaattagcaaagttagtcctggagcatttacacctttggtgaagttggaacgactttatctgtccaagaatcagctgaaggaattgccagaaaaaatgcccaaaactcttcaggagctgcgtgcccatgagaatgagatcaccaaagtgcgaaaagttactttcaatggactgaaccagatgattgtcatagaactgggcaccaatccgctgaagagctcaggaattgaaaatggggctttccagggaatgaagaagctctcctacatccgcattgctgataccaatatcaccagcattcctcaaggtcttcctccttcccttacggaattacatcttgatggcaacaaaatcagcagagttgatgcagctagcctgaaaggactgaataatttggctaagttgggattgagtttcaacagcatctctgctgttgacaatggctctctggccaacacgcctcatctgagggagcttcacttggacaacaacaagcttaccagagtacctggtgggctggcagagcataagtacatccaggttgtctaccttcataacaacaatatctctgtagttggatcaagtgacttctgcccacctggacacaacaccaaaaaggcttcttattcgggtgtgagtcttttcagcaacccggtccagtactgggagatacagccatccaccttcagatgtgtctacgtgcgctctgccattcaactcggaaactataagtga

SEQ ID NO: 29 - protein, 805 aa, Artificial Sequence
  synthetic
MMSFVSLLLVGILFHATQAEVQLVESGGGLVQPGGSLRLSCAASGFTFSRYWMSWVRQAPGKGLEWVANIKQDGSEKYYVDSVKGRFTISRDNAKNSLYLQMNSLRAEDTAVYYCAREGGWFGELAFDYWGQGTLVTVSSASTKGPSVFPLAPSSKSTSGGTAALGCLVKDYFPEPVTVSWNSGALTSGVHTFPAVLQSSGLYSLSSVVTVPSSSLGTQTYICNVNHKPSNTKVDKRVEPKSCDKTHTCPPCPAPEFEGGPSVFLFPPKPKDTLMISRTPEVTCVVVDVSHEDPEVKFNWYVDGVEVHNAKTKPREEQYNSTYRVVSVLTVLHQDWLNGKEYKCKVSNKALPASIEKTISKAKGQPREPQVYTLPPSREEMTKNQVSLTCLVKGFYPSDIAVEWESNGQPENNYKTTPPVLDSDGSFFLYSKLTVDKSRWQQGNVFSCSVMHEALHNHYTQKSLSLSPGKSGGGGSDEAAGIGPEVPDDRDFEPSLGPVCPFRCQCHLRVVQCSDLGLDKVPKDLPPDTTLLDLQNNKITEIKDGDFKNLKNLHALILVNNKISKVSPGAFTPLVKLERLYLSKNQLKELPEKMPKTLQELRAHENEITKVRKVTFNGLNQMIVIELGTNPLKSSGIENGAFQGMKKLSYIRIADTNITSIPQGLPPSLTELHLDGNKISRVDAASLKGLNNLAKLGLSFNSISAVDNGSLANTPHLRELHLDNNKLTRVPGGLAEHKYIQVVYLHNNNISVVGSSDFCPPGHNTKKASYSGVSLFSNPVQYWEIQPSTFRCVYVRSAIQLGNYK

SEQ ID NO: 30 - DNA, 705 bp, Artificial Sequence
  synthetic
atgatgtcctttgtctctctgctcctggttggcatcctattccatgccacccaggccgagatagttttgactcaaagccctggaacgctctctttgtctcccggcgagcgggcgaccctttcctgtagggctagccagagggtatcttcctcttacctggcatggtaccagcaaaagcccggacaagccccccgacttctgatttatgacgcctcatcccgggcgacaggcatccctgaccgattttcagggagtggctctggtaccgattttacgcttacgatttccaggctggagcccgaggatttcgcagtgtattactgtcaacaatacggcagcttgccctggacctttggacaaggaaccaaggtagagatcaaaaggaccgttgccgccccgtccgtgttcatcttccctccgagcgatgagcaacttaaaagtggaactgcaagcgttgtatgtcttctgaacaatttctatccccgagaagccaaggtacagtggaaagtggataatgccctccaatctggcaatagccaagagtctgtcacagagcaggacagcaaggactcaacttattcacttagctccaccctgacgctgagtaaagcagactacgagaagcataaggtgtatgcttgtgaggttacacaccaaggcttgtcttctcctgtcacgaagtctttcaataggggcgaatgctga

SEQ ID NO: 31 - protein, 234 aa, Artificial Sequence
  synthetic
MMSFVSLLLVGILFHATQAEIVLTQSPGTLSLSPGERATLSCRASQRVSSSYLAWYQQKPGQAPRLLIYDASSRATGIPDRFSGSGSGTDFTLTISRLEPEDFAVYYCQQYGSLPWTFGQGTKVEIKRTVAAPSVFIFPPSDEQLKSGTASVVCLLNNFYPREAKVQWKVDNALQSGNSQESVTEQDSKDSTYSLSSTLTLSKADYEKHKVYACEVTHQGLSSPVTKSFNRGEC

SEQ ID NO: 32 - protein, 451 aa, Artificial Sequence
  synthetic
EVQLVESGGGLVQPGGSLRLSCAASGFTFSRYWMSWVRQAPGKGLEWVANIKQDGSEKYYVDSVKGRFTISRDNAKNSLYLQMNSLRAEDTAVYYCAREGGWFGELAFDYWGQGTLVTVSSASTKGPSVFPLAPSSKSTSGGTAALGCLVKDYFPEPVTVSWNSGALTSGVHTFPAVLQSSGLYSLSSVVTVPSSSLGTQTYICNVNHKPSNTKVDKRVEPKSCDKTHTCPPCPAPEFEGGPSVFLFPPKPKDTLMISRTPEVTCVVVDVSHEDPEVKFNWYVDGVEVHNAKTKPREEQYNSTYRVVSVLTVLHQDWLNGKEYKCKVSNKALPASIEKTISKAKGQPREPQVYTLPPSREEMTKNQVSLTCLVKGFYPSDIAVEWESNGQPENNYKTTPPVLDSDGSFFLYSKLTVDKSRWQQGNVFSCSVMHEALHNHYTQKSLSLSPGK

SEQ ID NO: 33 - protein, 215 aa, Artificial Sequence
  synthetic
EIVLTQSPGTLSLSPGERATLSCRASQRVSSSYLAWYQQKPGQAPRLLIYDASSRATGIPDRFSGSGSGTDFTLTISRLEPEDFAVYYCQQYGSLPWTFGQGTKVEIKRTVAAPSVFIFPPSDEQLKSGTASVVCLLNNFYPREAKVQWKVDNALQSGNSQESVTEQDSKDSTYSLSSTLTLSKADYEKHKVYACEVTHQGLSSPVTKSFNRGEC

SEQ ID NO: 34 - DNA, 2385 bp, Artificial Sequence
  synthetic
atgatgtcctttgtctctctgctcctggttggcatcctattccatgccacccaggcccaagtccagctcgtggaatcaggagggggtgtagtccaaccagggcggagcctccgacttgattgtaaagcatcaggaattacattttctaatagcggaatgcattgggtccgacaagcgccaggcaagggactggaatgggtcgcggtgatatggtatgatggatcaaaacgctattatgcggactctgtgaagggtcgattcactattagcagagataacagcaagaatactctcttccttcagatgaattcacttagggcagaggacacagcggtgtactattgcgcgacgaacgacgattattggggccaagggacattggtaacggtgagttctgctagtactaaagggccttccgtcttcccactcgccccttgttctagaagtactagtgagtcaacagctgctttgggttgcttggttaaagactactttcctgaacccgtgactgtgtcttggaattccggtgctcttacttcaggtgttcatacattcccagcagtattgcagagctctggcttgtattctctctcctcagtggtgacagtaccttcctcctctcttggcacaaaaacttacacatgtaatgtagaccataaaccatcaaacacgaaagttgacaagagagtagaaagcaagtatgggcctccatgtcccccgtgcccggcgcccgagttcctgggtggtccgtcagtgttcttgttccctcccaagccaaaagatacattgatgataagtcggacgccggaggtcacatgtgtagtagttgatgtctctcaggaggatcctgaggtgcagtttaactggtacgtcgatggtgttgaggtacacaacgccaaaactaagccgagggaagagcagttcaattcaacatatcgggtcgtgtccgtattgacagttctgcaccaagattggttgaacggaaaagagtataagtgcaaagttagcaataagggacttccgtcctcaattgaaaaaaccatttccaaagcgaaaggccaacctcgggaacctcaggtatataccttgccacccagccaagaagaaatgactaaaaaccaggttagtttgacatgtttggttaaaggcttttacccgtccgacattgccgtcgagtgggaaagcaatgggcagcctgaaaataactacaagacaaccccaccagtattggattccgacggttccttctttctttacagccgcctcaccgtcgataagagtcggtggcaagaggggaatgtcttttcctgtagtgtcatgcacgaagcacttcacaaccattacacccaaaaatcattgtccctgtcactggggaaatccgggggtggcggatccgatgaggctgcagggataggcccagaagttcctgatgaccgcgacttcgagccctccctaggcccagtgtgccccttccgctgtcaatgccatcttcgagtggtccagtgttctgatttgggtctggacaaagtgccaaaggatcttccccctgacacaactctgctagacctgcaaaacaacaaaataaccgaaatcaaagatggagactttaagaacctgaagaaccttcacgcattgattcttgtcaacaataaaattagcaaagttagtcctggagcatttacacctttggtgaagttggaacgactttatctgtccaagaatcagctgaaggaattgccagaaaaaatgcccaaaactcttcaggagctgcgtgcccatgagaatgagatcaccaaagtgcgaaaagttactttcaatggactgaaccagatgattgtcatagaactgggcaccaatccgctgaagagctcaggaattgaaaatggggctttccagggaatgaagaagctctcctacatccgcattgctgataccaatatcaccagcattcctcaaggtcttcctccttcccttacggaattacatcttgatggcaacaaaatcagcagagttgatgcagctagcctgaaaggactgaataatttggctaagttgggattgagtttcaacagcatctctgctgttgacaatggctctctggccaacacgcctcatctgagggagcttcacttggacaacaacaagcttaccagagtacctggtgggctggcagagcataagtacatccaggttgtctaccttcataacaacaatatctctgtagttggatcaagtgacttctgcccacctggacacaacaccaaaaaggcttcttattcgggtgtgagtcttttcagcaacccggtccagtactgggagatacagccatccaccttcagatgtgtctacgtgcgctctgccattcaactcggaaactataagtga

SEQ ID NO: 35 - protein, 794 aa, Artificial Sequence
  synthetic
MMSFVSLLLVGILFHATQAQVQLVESGGGVVQPGRSLRLDCKASGITFSNSGMHWVRQAPGKGLEWVAVIWYDGSKRYYADSVKGRFTISRDNSKNTLFLQMNSLRAEDTAVYYCATNDDYWGQGTLVTVSSASTKGPSVFPLAPCSRSTSESTAALGCLVKDYFPEPVTVSWNSGALTSGVHTFPAVLQSSGLYSLSSVVTVPSSSLGTKTYTCNVDHKPSNTKVDKRVESKYGPPCPPCPAPEFLGGPSVFLFPPKPKDTLMISRTPEVTCVVVDVSQEDPEVQFNWYVDGVEVHNAKTKPREEQFNSTYRVVSVLTVLHQDWLNGKEYKCKVSNKGLPSSIEKTISKAKGQPREPQVYTLPPSQEEMTKNQVSLTCLVKGFYPSDIAVEWESNGQPENNYKTTPPVLDSDGSFFLYSRLTVDKSRWQEGNVFSCSVMHEALHNHYTQKSLSLSLGKSGGGGSDEAAGIGPEVPDDRDFEPSLGPVCPFRCQCHLRVVQCSDLGLDKVPKDLPPDTTLLDLQNNKITEIKDGDFKNLKNLHALILVNNKISKVSPGAFTPLVKLERLYLSKNQLKELPEKMPKTLQELRAHENEITKVRKVTFNGLNQMIVIELGTNPLKSSGIENGAFQGMKKLSYIRIADTNITSIPQGLPPSLTELHLDGNKISRVDAASLKGLNNLAKLGLSFNSISAVDNGSLANTPHLRELHLDNNKLTRVPGGLAEHKYIQVVYLHNNNISVVGSSDFCPPGHNTKKASYSGVSLFSNPVQYWEIQPSTFRCVYVRSAIQLGNYK

SEQ ID NO: 36 - DNA, 702 bp, Artificial Sequence
  synthetic
atgatgtcctttgtctctctgctcctggttggcatcctattccatgccacccaggccgaaatcgtattgactcagtcccctgctacactttcactgagtccgggtgagcgggcgactttgtcatgtcgggcatcacagagtgtaagtagttatctggcctggtatcaacagaaaccgggacaggctcctcgcctgctgatttatgacgcaagcaatcgcgcgaccggcatcccggcgaggttctcagggtctggatcaggtactgactttacccttacgatctcttctctcgaacctgaggatttcgctgtctattactgccagcagtcttctaactggccgagaacatttggtcaagggacaaaagtcgagattaagcgaactgtcgcagcgccatctgtctttatcttccctccaagcgacgaacagcttaagagtggcaccgccagtgttgtctgccttctgaataacttctatccaagggaagcgaaagttcagtggaaggtggataacgctctgcagtctgggaactctcaggaaagtgtaacagaacaagactccaaagactcaacctactctcttagttccacgttgaccctctccaaagcggactatgagaagcataaggtctacgcttgcgaggtaacacaccaggggctgagtagtccggttacgaagagcttcaacagaggggaatgctga

SEQ ID NO: 37 - protein, 233 aa, Artificial Sequence
  synthetic
MMSFVSLLLVGILFHATQAEIVLTQSPATLSLSPGERATLSCRASQSVSSYLAWYQQKPGQAPRLLIYDASNRATGIPARFSGSGSGTDFTLTISSLEPEDFAVYYCQQSSNWPRTFGQGTKVEIKRTVAAPSVFIFPPSDEQLKSGTASVVCLLNNFYPREAKVQWKVDNALQSGNSQESVTEQDSKDSTYSLSSTLTLSKADYEKHKVYACEVTHQGLSSPVTKSFNRGEC

SEQ ID NO: 38 - protein, 440 aa, Artificial Sequence
  synthetic
QVQLVESGGGVVQPGRSLRLDCKASGITFSNSGMHWVRQAPGKGLEWVAVIWYDGSKRYYADSVKGRFTISRDNSKNTLFLQMNSLRAEDTAVYYCATNDDYWGQGTLVTVSSASTKGPSVFPLAPCSRSTSESTAALGCLVKDYFPEPVTVSWNSGALTSGVHTFPAVLQSSGLYSLSSVVTVPSSSLGTKTYTCNVDHKPSNTKVDKRVESKYGPPCPPCPAPEFLGGPSVFLFPPKPKDTLMISRTPEVTCVVVDVSQEDPEVQFNWYVDGVEVHNAKTKPREEQFNSTYRVVSVLTVLHQDWLNGKEYKCKVSNKGLPSSIEKTISKAKGQPREPQVYTLPPSQEEMTKNQVSLTCLVKGFYPSDIAVEWESNGQPENNYKTTPPVLDSDGSFFLYSRLTVDKSRWQEGNVFSCSVMHEALHNHYTQKSLSLSLGK

SEQ ID NO: 39 - protein, 214 aa, Artificial Sequence
  synthetic
EIVLTQSPATLSLSPGERATLSCRASQSVSSYLAWYQQKPGQAPRLLIYDASNRATGIPARFSGSGSGTDFTLTISSLEPEDFAVYYCQQSSNWPRTFGQGTKVEIKRTVAAPSVFIFPPSDEQLKSGTASVVCLLNNFYPREAKVQWKVDNALQSGNSQESVTEQDSKDSTYSLSSTLTLSKADYEKHKVYACEVTHQGLSSPVTKSFNRGEC

SEQ ID NO: 40 - DNA, 2406 bp, Artificial Sequence
  synthetic
atgatgtcctttgtctctctgctcctggttggcatcctattccatgccacccaggcccaggtgcaattggtccaaagtggggtcgaggtcaagaagccaggagcttctgtaaaagtttcatgtaaggcatctgggtataccttcacgaactactatatgtattgggtgcgccaagcgccagggcagggcctcgaatggatgggtggcatcaatccgagcaacgggggcaccaactttaacgaaaagtttaaaaaccgggtcaccttgacaacggacagtagcacgactaccgcttatatggagctgaagagtttgcagtttgatgatactgcggtttattattgtgcacgcagagattataggttcgacatgggcttcgactactggggtcaaggtactacggtaactgtatcatctgctagtacaaagggcccttccgttttccccctcgccccgtgcagccgctcaacgtccgaaagcaccgctgcacttgggtgccttgtaaaagactattttccagagccagttaccgtgtcttggaatagtggcgcacttacgtccggggtgcacacttttccggctgtcttgcaatcctctggactctattccttgagtagcgtcgtaacagtaccaagtagtagtctcggcaccaaaacgtatacgtgcaatgttgatcataagcctagcaacacgaaagttgacaaaagagttgagagtaaatatggacccccctgtccgccatgcccggcccctgaattccttgggggcccgtctgtatttcttttcccgcccaagccgaaggatacactgatgataagcagaacgcctgaggttacctgcgtcgtggtcgacgtaagccaggaagatcctgaggtgcaatttaattggtatgtggacggggtcgaggttcataatgcaaaaacaaaaccccgagaggagcaatttaattcaacgtacagagtcgttagcgtacttacagtgctgcaccaggattggctcaacgggaaggagtataagtgcaaggtgtctaataaaggtttgccctccagtatagaaaaaaccatctcaaaggcgaaaggacagcctagagaacctcaagtatataccctcccaccctcccaagaagagatgacaaagaaccaagtgagtctcacatgcctcgtcaagggtttctacccaagcgatatagccgtagagtgggaatcaaatggtcagccggagaataactacaaaactactccgccagtcttggatagcgacgggtcttttttcctgtactctaggctgacggtggacaagtcaagatggcaggaaggaaatgtttttagctgctccgttatgcatgaggctctccacaatcattatacacaaaaaagtttgtctctgtcattggggaaatccgggggtggcggatccgatgaggctgcagggataggcccagaagttcctgatgaccgcgacttcgagccctccctaggcccagtgtgccccttccgctgtcaatgccatcttcgagtggtccagtgttctgatttgggtctggacaaagtgccaaaggatcttccccctgacacaactctgctagacctgcaaaacaacaaaataaccgaaatcaaagatggagactttaagaacctgaagaaccttcacgcattgattcttgtcaacaataaaattagcaaagttagtcctggagcatttacacctttggtgaagttggaacgactttatctgtccaagaatcagctgaaggaattgccagaaaaaatgcccaaaactcttcaggagctgcgtgcccatgagaatgagatcaccaaagtgcgaaaagttactttcaatggactgaaccagatgattgtcatagaactgggcaccaatccgctgaagagctcaggaattgaaaatggggctttccagggaatgaagaagctctcctacatccgcattgctgataccaatatcaccagcattcctcaaggtcttcctccttcccttacggaattacatcttgatggcaacaaaatcagcagagttgatgcagctagcctgaaaggactgaataatttggctaagttgggattgagtttcaacagcatctctgctgttgacaatggctctctggccaacacgcctcatctgagggagcttcacttggacaacaacaagcttaccagagtacctggtgggctggcagagcataagtacatccaggttgtctaccttcataacaacaatatctctgtagttggatcaagtgacttctgcccacctggacacaacaccaaaaaggcttcttattcgggtgtgagtcttttcagcaacccggtccagtactgggagatacagccatccaccttcagatgtgtctacgtgcgctctgccattcaactcggaaactataagtga

SEQ ID NO: 41 - protein, 801 aa, Artificial Sequence
  synthetic
MMSFVSLLLVGILFHATQAQVQLVQSGVEVKKPGASVKVSCKASGYTFTNYYMYWVRQAPGQGLEWMGGINPSNGGTNFNEKFKNRVTLTTDSSTTTAYMELKSLQFDDTAVYYCARRDYRFDMGFDYWGQGTTVTVSSASTKGPSVFPLAPCSRSTSESTAALGCLVKDYFPEPVTVSWNSGALTSGVHTFPAVLQSSGLYSLSSVVTVPSSSLGTKTYTCNVDHKPSNTKVDKRVESKYGPPCPPCPAPEFLGGPSVFLFPPKPKDTLMISRTPEVTCVVVDVSQEDPEVQFNWYVDGVEVHNAKTKPREEQFNSTYRVVSVLTVLHQDWLNGKEYKCKVSNKGLPSSIEKTISKAKGQPREPQVYTLPPSQEEMTKNQVSLTCLVKGFYPSDIAVEWESNGQPENNYKTTPPVLDSDGSFFLYSRLTVDKSRWQEGNVFSCSVMHEALHNHYTQKSLSLSLGKSGGGGSDEAAGIGPEVPDDRDFEPSLGPVCPFRCQCHLRVVQCSDLGLDKVPKDLPPDTTLLDLQNNKITEIKDGDFKNLKNLHALILVNNKISKVSPGAFTPLVKLERLYLSKNQLKELPEKMPKTLQELRAHENEITKVRKVTFNGLNQMIVIELGTNPLKSSGIENGAFQGMKKLSYIRIADTNITSIPQGLPPSLTELHLDGNKISRVDAASLKGLNNLAKLGLSFNSISAVDNGSLANTPHLRELHLDNNKLTRVPGGLAEHKYIQVVYLHNNNISVVGSSDFCPPGHNTKKASYSGVSLFSNPVQYWEIQPSTFRCVYVRSAIQLGNYK

SEQ ID NO: 42 - DNA, 714 bp, Artificial Sequence
  synthetic
atgatgtcctttgtctctctgctcctggttggcatcctattccatgccacccaggccgaaattgttcttacgcagagtccagcaactttgtcactctctcccggcgaacgagcgacattgtcctgtcgcgcgagtaagggtgtctcaacatctggatactcatatctgcattggtaccagcaaaaaccgggacaagcgccgcgattgctgatttatctcgcctcctaccttgaaagtggtgtgcctgcgaggttctccggtagtggatcaggcaccgatttcactttgaccatcagcagcctcgaaccagaagattttgccgtctactactgccaacatagcagggatttgccactgacattcggcgggggtacgaaagttgagattaaacggactgtagcggcaccttctgtcttcatcttcccaccaagcgatgagcagcttaaaagcggtacagcttcagtggtgtgccttttgaacaacttttatccgcgagaagccaaggtccaatggaaggtggataacgctttgcaatccggtaactcacaggagtcagtaacagagcaagatagtaaagatagcacgtattcacttagcagtacccttactcttagcaaggctgattatgaaaaacataaggtatatgcgtgcgaggtaacgcaccaaggacttagctccccagtgacgaagtcatttaaccggggggagtgctga

SEQ ID NO: 43 - protein, 237 aa, Artificial Sequence
  synthetic
MMSFVSLLLVGILFHATQAEIVLTQSPATLSLSPGERATLSCRASKGVSTSGYSYLHWYQQKPGQAPRLLIYLASYLESGVPARFSGSGSGTDFTLTISSLEPEDFAVYYCQHSRDLPLTFGGGTKVEIKRTVAAPSVFIFPPSDEQLKSGTASVVCLLNNFYPREAKVQWKVDNALQSGNSQESVTEQDSKDSTYSLSSTLTLSKADYEKHKVYACEVTHQGLSSPVTKSFNRGEC

SEQ ID NO: 44 - protein, 447 aa, Artificial Sequence
  synthetic
QVQLVQSGVEVKKPGASVKVSCKASGYTFTNYYMYWVRQAPGQGLEWMGGINPSNGGTNFNEKFKNRVTLTTDSSTTTAYMELKSLQFDDTAVYYCARRDYRFDMGFDYWGQGTTVTVSSASTKGPSVFPLAPCSRSTSESTAALGCLVKDYFPEPVTVSWNSGALTSGVHTFPAVLQSSGLYSLSSVVTVPSSSLGTKTYTCNVDHKPSNTKVDKRVESKYGPPCPPCPAPEFLGGPSVFLFPPKPKDTLMISRTPEVTCVVVDVSQEDPEVQFNWYVDGVEVHNAKTKPREEQFNSTYRVVSVLTVLHQDWLNGKEYKCKVSNKGLPSSIEKTISKAKGQPREPQVYTLPPSQEEMTKNQVSLTCLVKGFYPSDIAVEWESNGQPENNYKTTPPVLDSDGSFFLYSRLTVDKSRWQEGNVFSCSVMHEALHNHYTQKSLSLSLGK

SEQ ID NO: 45 - protein, 218 aa, Artificial Sequence
  synthetic
EIVLTQSPATLSLSPGERATLSCRASKGVSTSGYSYLHWYQQKPGQAPRLLIYLASYLESGVPARFSGSGSGTDFTLTISSLEPEDFAVYYCQHSRDLPLTFGGGTKVEIKRTVAAPSVFIFPPSDEQLKSGTASVVCLLNNFYPREAKVQWKVDNALQSGNSQESVTEQDSKDSTYSLSSTLTLSKADYEKHKVYACEVTHQGLSSPVTKSFNRGEC

SEQ ID NO: 46 - protein, 329 aa, Artificial Sequence; identical to SEQ ID NO: 7
  synthetic

SEQ ID NO: 47 - protein, 14 aa, Artificial Sequence
  synthetic
GPFQQRGLFDFMLE

SEQ ID NO: 48 - DNA, 42 bp, Artificial Sequence
  synthetic
ggcccgtttcaacagagaggcttatttgactttatgctagaa

SEQ ID NO: 49 - DNA, 990 bp, Artificial Sequence
  synthetic
gatgaggctgcagggataggcccagaagttcctgatgaccgcgacttcgagccctccctaggcccagtgtgccccttccgctgtcaatgccatcttcgagtggtccagtgttctgatttgggtctggacaaagtgccaaaggatcttccccctgacacaactctgctagacctgcaaaacaacaaaataaccgaaatcaaagatggagactttaagaacctgaagaaccttcacgcattgattcttgtcaacaataaaattagcaaagttagtcctggagcatttacacctttggtgaagttggaacgactttatctgtccaagaatcagctgaaggaattgccagaaaaaatgcccaaaactcttcaggagctgcgtgcccatgagaatgagatcaccaaagtgcgaaaagttactttcaatggactgaaccagatgattgtcatagaactgggcaccaatccgctgaagagctcaggaattgaaaatggggctttccagggaatgaagaagctctcctacatccgcattgctgataccaatatcaccagcattcctcaaggtcttcctccttcccttacggaattacatcttgatggcaacaaaatcagcagagttgatgcagctagcctgaaaggactgaataatttggctaagttgggattgagtttcaacagcatctctgctgttgacaatggctctctggccaacacgcctcatctgagggagcttcacttggacaacaacaagcttaccagagtacctggtgggctggcagagcataagtacatccaggttgtctaccttcataacaacaatatctctgtagttggatcaagtgacttctgcccacctggacacaacaccaaaaaggcttcttattcgggtgtgagtcttttcagcaacccggtccagtactgggagatacagccatccaccttcagatgtgtctacgtgcgctctgccattcaactcggaaactataagtga

SEQ ID NO: 50 - DNA, 2415 bp, Artificial Sequence; identical to SEQ ID NO: 22
  synthetic

SEQ ID NO: 51 - protein, 804 aa, Artificial Sequence; identical to SEQ ID NO: 23
  synthetic

SEQ ID NO: 52 - DNA, 708 bp, Artificial Sequence; identical to SEQ ID NO: 24
  synthetic

SEQ ID NO: 53 - protein, 235 aa, Artificial Sequence; identical to SEQ ID NO: 25
  synthetic

SEQ ID NO: 54 - DNA, 3420 bp, Artificial Sequence
  synthetic
atgatgtcctttgtctctctgctcctggttggcatcctattccatgccacccaggccgaggtacagcttttggagtcaggcggggggctcgtccaacctggggggtcactccggttgtcatgtgctgccagtggcttcacattctcatcttacattatgatgtgggttcgacaggcccctgggaaggggctggagtgggtttcctccatctacccctccgggggaattaccttctatgccgacacggtaaagggtcgcttcactataagtcgagataacagcaaaaatacgctgtatctccagatgaactctctcagggctgaggacacagctgtatattactgcgcgcggattaagttggggaccgtcacaacagtggattactggggtcaaggcactctggtaaccgtatcctcagcatccaccaagggcccaagtgtattcccgctggccccttcaagtaaatccacgtctggcggcacagccgctctcggttgcctggttaaggactacttcccagaacctgtcactgtcagttggaactcaggcgcattgacatctggtgtccatacattccccgcagtcctgcaaagctctggactttacagtcttagtagcgtagtgacagtcccatcttcaagtcttgggacccaaacttatatttgcaacgtaaatcataaaccctccaacactaaagtagacaaaaaagtagagccgaaatcttgcgacaaaacgcatacatgcccaccatgtcccgctccggaactcctgggcggcccgtccgtttttctctttcccccaaagcccaaggatacgcttatgatcagcagaacaccggaagttacttgtgtagtcgttgacgtgtctcacgaagatcccgaagtcaaatttaattggtatgtggatggcgtcgaagtgcacaacgcaaaaaccaaacccagagaggaacagtataacagcacgtatcgagtggtctccgtacttacggtcctccaccaggactggttgaatggcaaggagtacaagtgcaaagtgagcaataaagcgttgccagccccgatcgaaaaaaccatcagcaaggccaagggacagcctagagagccgcaggtttacaccttgccgccatcaagggatgaactgactaaaaaccaggtatccctgacctgcctggttaagggtttttaccccagtgatatagcggttgaatgggagtctaacgggcagccagagaacaactacaaaacgacacctcccgttctggattccgatggcagctttttcttgtattctaaactcaccgtggataaatcccgatggcagcaaggcaacgtcttctcctgcagcgtgatgcatgaagccttgcacaaccactatacccaaaagagtctcagcctgtcacccgggaaatccgggggtggcggatccgatgaggctgcagggataggcccagaagttcctgatgaccgcgacttcgagccctccctaggcccagtgtgccccttccgctgtcaatgccatcttcgagtggtccagtgttctgatttgggtctggacaaagtgccaaaggatcttccccctgacacaactctgctagacctgcaaaacaacaaaataaccgaaatcaaagatggagactttaagaacctgaagaaccttcacgcattgattcttgtcaacaataaaattagcaaagttagtcctggagcatttacacctttggtgaagttggaacgactttatctgtccaagaatcagctgaaggaattgccagaaaaaatgcccaaaactcttcaggagctgcgtgcccatgagaatgagatcaccaaagtgcgaaaagttactttcaatggactgaaccagatgattgtcatagaactgggcaccaatccgctgaagagctcaggaattgaaaatggggctttccagggaatgaagaagctctcctacatccgcattgctgataccaatatcaccagcattcctcaaggtcttcctccttcccttacggaattacatcttgatggcaacaaaatcagcagagttgatgcagctagcctgaaaggactgaataatttggctaagttgggattgagtttcaacagcatctctgctgttgacaatggctctctggccaacacgcctcatctgagggagcttcacttggacaacaacaagcttaccagagtacctggtgggctggcagagcataagtacatccaggttgtctaccttcataacaacaatatctctgtagttggatcaagtgacttctgcccacctggacacaacaccaaaaaggcttcttattcgggtgtgagtcttttcagcaacccggtccagtactgggagatacagccatccaccttcagatgtgtctacgtgcgctctgccattcaactcggaaactataagtccgggggtggcggatccgatgaggctgcagggataggcccagaagttcctgatgaccgcgacttcgagccctccctaggcccagtgtgccccttccgctgtcaatgccatcttcgagtggtccagtgttctgatttgggtctggacaaagtgccaaaggatcttccccctgacacaactctgctagacctgcaaaacaacaaaataaccgaaatcaaagatggagactttaagaacctgaagaaccttcacgcattgattcttgtcaacaataaaattagcaaagttagtcctggagcatttacacctttggtgaagttggaacgactttatctgtccaagaatcagctgaaggaattgccagaaaaaatgcccaaaactcttcaggagctgcgtgcccatgagaatgagatcaccaaagtgcgaaaagttactttcaatggactgaaccagatgattgtcatagaactgggcaccaatccgctgaagagctcaggaattgaaaatggggctttccagggaatgaagaagctctcctacatccgcattgctgataccaatatcaccagcattcctcaaggtcttcctccttcccttacggaattacatcttgatggcaacaaaatcagcagagttgatgcagctagcctgaaaggactgaataatttggctaagttgggattgagtttcaacagcatctctgctgttgacaatggctctctggccaacacgcctcatctgagggagcttcacttggacaacaacaagcttaccagagtacctggtgggctggcagagcataagtacatccaggttgtctaccttcataacaacaatatctctgtagttggatcaagtgacttctgcccacctggacacaacaccaaaaaggcttcttattcgggtgtgagtcttttcagcaacccggtccagtactgggagatacagccatccaccttcagatgtgtctacgtgcgctctgccattcaactcggaaactataagtga

SEQ ID NO: 55 - protein, 1139 aa, Artificial Sequence
  synthetic
MMSFVSLLLVGILFHATQAEVQLLESGGGLVQPGGSLRLSCAASGFTFSSYIMMWVRQAPGKGLEWVSSIYPSGGITFYADTVKGRFTISRDNSKNTLYLQMNSLRAEDTAVYYCARIKLGTVTTVDYWGQGTLVTVSSASTKGPSVFPLAPSSKSTSGGTAALGCLVKDYFPEPVTVSWNSGALTSGVHTFPAVLQSSGLYSLSSVVTVPSSSLGTQTYICNVNHKPSNTKVDKKVEPKSCDKTHTCPPCPAPELLGGPSVFLFPPKPKDTLMISRTPEVTCVVVDVSHEDPEVKFNWYVDGVEVHNAKTKPREEQYNSTYRVVSVLTVLHQDWLNGKEYKCKVSNKALPAPIEKTISKAKGQPREPQVYTLPPSRDELTKNQVSLTCLVKGFYPSDIAVEWESNGQPENNYKTTPPVLDSDGSFFLYSKLTVDKSRWQQGNVFSCSVMHEALHNHYTQKSLSLSPGKSGGGGSDEAAGIGPEVPDDRDFEPSLGPVCPFRCQCHLRVVQCSDLGLDKVPKDLPPDTTLLDLQNNKITEIKDGDFKNLKNLHALILVNNKISKVSPGAFTPLVKLERLYLSKNQLKELPEKMPKTLQELRAHENEITKVRKVTFNGLNQMIVIELGTNPLKSSGIENGAFQGMKKLSYIRIADTNITSIPQGLPPSLTELHLDGNKISRVDAASLKGLNNLAKLGLSFNSISAVDNGSLANTPHLRELHLDNNKLTRVPGGLAEHKYIQVVYLHNNNISVVGSSDFCPPGHNTKKASYSGVSLFSNPVQYWEIQPSTFRCVYVRSAIQLGNYKSGGGGSDEAAGIGPEVPDDRDFEPSLGPVCPFRCQCHLRVVQCSDLGLDKVPKDLPPDTTLLDLQNNKITEIKDGDFKNLKNLHALILVNNKISKVSPGAFTPLVKLERLYLSKNQLKELPEKMPKTLQELRAHENEITKVRKVTFNGLNQMIVIELGTNPLKSSGIENGAFQGMKKLSYIRIADTNITSIPQGLPPSLTELHLDGNKISRVDAASLKGLNNLAKLGLSFNSISAVDNGSLANTPHLRELHLDNNKLTRVPGGLAEHKYIQVVYLHNNNISVVGSSDFCPPGHNTKKASYSGVSLFSNPVQYWEIQPSTFRCVYVRSAIQLGNYK

SEQ ID NO: 56 - DNA, 2373 bp, Artificial Sequence
  synthetic
atgatgtcctttgtctctctgctcctggttggcatcctattccatgccacccaggccgaggtacagcttttggagtcaggcggggggctcgtccaacctggggggtcactccggttgtcatgtgctgccagtggcttcacattctcatcttacattatgatgtgggttcgacaggcccctgggaaggggctggagtgggtttcctccatctacccctccgggggaattaccttctatgccgacacggtaaagggtcgcttcactataagtcgagataacagcaaaaatacgctgtatctccagatgaactctctcagggctgaggacacagctgtatattactgcgcgcggattaagttggggaccgtcacaacagtggattactggggtcaaggcactctggtaaccgtatcctcagcatccaccaagggcccaagtgtattcccgctggccccttcaagtaaatccacgtctggcggcacagccgctctcggttgcctggttaaggactacttcccagaacctgtcactgtcagttggaactcaggcgcattgacatctggtgtccatacattccccgcagtcctgcaaagctctggactttacagtcttagtagcgtagtgacagtcccatcttcaagtcttgggacccaaacttatatttgcaacgtaaatcataaaccctccaacactaaagtagacaaaaaagtagagccgaaatcttgcgacaaaacgcatacatgcccaccatgtcccgctccggaactcctgggcggcccgtccgtttttctctttcccccaaagcccaaggatacgcttatgatcagcagaacaccggaagttacttgtgtagtcgttgacgtgtctcacgaagatcccgaagtcaaatttaattggtatgtggatggcgtcgaagtgcacaacgcaaaaaccaaacccagagaggaacagtataacagcacgtatcgagtggtctccgtacttacggtcctccaccaggactggttgaatggcaaggagtacaagtgcaaagtgagcaataaagcgttgccagccccgatcgaaaaaaccatcagcaaggccaagggacagcctagagagccgcaggtttacaccttgccgccatcaagggatgaactgactaaaaaccaggtatccctgacctgcctggttaagggtttttaccccagtgatatagcggttgaatgggagtctaacgggcagccagagaacaactacaaaacgacacctcccgttctggattccgatggcagctttttcttgtattctaaactcaccgtggataaatcccgatggcagcaaggcaacgtcttctcctgcagcgtgatgcatgaagccttgcacaaccactatacccaaaagagtctcagcctgtcacccgggaaatccgggggtggcggatccgacttcgagccctccctaggcccagtgtgccccttccgctgtcaatgccatcttcgagtggtccagtgttctgatttgggtctggacaaagtgccaaaggatcttccccctgacacaactctgctagacctgcaaaacaacaaaataaccgaaatcaaagatggagactttaagaacctgaagaaccttcacgcattgattcttgtcaacaataaaattagcaaagttagtcctggagcatttacacctttggtgaagttggaacgactttatctgtccaagaatcagctgaaggaattgccagaaaaaatgcccaaaactcttcaggagctgcgtgcccatgagaatgagatcaccaaagtgcgaaaagttactttcaatggactgaaccagatgattgtcatagaactgggcaccaatccgctgaagagctcaggaattgaaaatggggctttccagggaatgaagaagctctcctacatccgcattgctgataccaatatcaccagcattcctcaaggtcttcctccttcccttacggaattacatcttgatggcaacaaaatcagcagagttgatgcagctagcctgaaaggactgaataatttggctaagttgggattgagtttcaacagcatctctgctgttgacaatggctctctggccaacacgcctcatctgagggagcttcacttggacaacaacaagcttaccagagtacctggtgggctggcagagcataagtacatccaggttgtctaccttcataacaacaatatctctgtagttggatcaagtgacttctgcccacctggacacaacaccaaaaaggcttcttattcgggtgtgagtcttttcagcaacccggtccagtactgggagatacagccatccaccttcagatgtgtctacgtgcgctctgccattcaactcggaaactataagtga

SEQ ID NO: 57 - protein, 790 aa, Artificial Sequence
  synthetic
MMSFVSLLLVGILFHATQAEVQLLESGGGLVQPGGSLRLSCAASGFTFSSYIMMWVRQAPGKGLEWVSSIYPSGGITFYADTVKGRFTISRDNSKNTLYLQMNSLRAEDTAVYYCARIKLGTVTTVDYWGQGTLVTVSSASTKGPSVFPLAPSSKSTSGGTAALGCLVKDYFPEPVTVSWNSGALTSGVHTFPAVLQSSGLYSLSSVVTVPSSSLGTQTYICNVNHKPSNTKVDKKVEPKSCDKTHTCPPCPAPELLGGPSVFLFPPKPKDTLMISRTPEVTCVVVDVSHEDPEVKFNWYVDGVEVHNAKTKPREEQYNSTYRVVSVLTVLHQDWLNGKEYKCKVSNKALPAPIEKTISKAKGQPREPQVYTLPPSRDELTKNQVSLTCLVKGFYPSDIAVEWESNGQPENNYKTTPPVLDSDGSFFLYSKLTVDKSRWQQGNVFSCSVMHEALHNHYTQKSLSLSPGKSGGGGSDFEPSLGPVCPFRCQCHLRVVQCSDLGLDKVPKDLPPDTTLLDLQNNKITEIKDGDFKNLKNLHALILVNNKISKVSPGAFTPLVKLERLYLSKNQLKELPEKMPKTLQELRAHENEITKVRKVTFNGLNQMIVIELGTNPLKSSGIENGAFQGMKKLSYIRIADTNITSIPQGLPPSLTELHLDGNKISRVDAASLKGLNNLAKLGLSFNSISAVDNGSLANTPHLRELHLDNNKLTRVPGGLAEHKYIQVVYLHNNNISVVGSSDFCPPGHNTKKASYSGVSLFSNPVQYWEIQPSTFRCVYVRSAIQLGNYK

SEQ ID NO: 58 - DNA, 3336 bp, Artificial Sequence
  synthetic
atgatgtcctttgtctctctgctcctggttggcatcctattccatgccacccaggccgaggtacagcttttggagtcaggcggggggctcgtccaacctggggggtcactccggttgtcatgtgctgccagtggcttcacattctcatcttacattatgatgtgggttcgacaggcccctgggaaggggctggagtgggtttcctccatctacccctccgggggaattaccttctatgccgacacggtaaagggtcgcttcactataagtcgagataacagcaaaaatacgctgtatctccagatgaactctctcagggctgaggacacagctgtatattactgcgcgcggattaagttggggaccgtcacaacagtggattactggggtcaaggcactctggtaaccgtatcctcagcatccaccaagggcccaagtgtattcccgctggccccttcaagtaaatccacgtctggcggcacagccgctctcggttgcctggttaaggactacttcccagaacctgtcactgtcagttggaactcaggcgcattgacatctggtgtccatacattccccgcagtcctgcaaagctctggactttacagtcttagtagcgtagtgacagtcccatcttcaagtcttgggacccaaacttatatttgcaacgtaaatcataaaccctccaacactaaagtagacaaaaaagtagagccgaaatcttgcgacaaaacgcatacatgcccaccatgtcccgctccggaactcctgggcggcccgtccgtttttctctttcccccaaagcccaaggatacgcttatgatcagcagaacaccggaagttacttgtgtagtcgttgacgtgtctcacgaagatcccgaagtcaaatttaattggtatgtggatggcgtcgaagtgcacaacgcaaaaaccaaacccagagaggaacagtataacagcacgtatcgagtggtctccgtacttacggtcctccaccaggactggttgaatggcaaggagtacaagtgcaaagtgagcaataaagcgttgccagccccgatcgaaaaaaccatcagcaaggccaagggacagcctagagagccgcaggtttacaccttgccgccatcaagggatgaactgactaaaaaccaggtatccctgacctgcctggttaagggtttttaccccagtgatatagcggttgaatgggagtctaacgggcagccagagaacaactacaaaacgacacctcccgttctggattccgatggcagctttttcttgtattctaaactcaccgtggataaatcccgatggcagcaaggcaacgtcttctcctgcagcgtgatgcatgaagccttgcacaaccactatacccaaaagagtctcagcctgtcacccgggaaatccgggggtggcggatccgacttcgagccctccctaggcccagtgtgccccttccgctgtcaatgccatcttcgagtggtccagtgttctgatttgggtctggacaaagtgccaaaggatcttccccctgacacaactctgctagacctgcaaaacaacaaaataaccgaaatcaaagatggagactttaagaacctgaagaaccttcacgcattgattcttgtcaacaataaaattagcaaagttagtcctggagcatttacacctttggtgaagttggaacgactttatctgtccaagaatcagctgaaggaattgccagaaaaaatgcccaaaactcttcaggagctgcgtgcccatgagaatgagatcaccaaagtgcgaaaagttactttcaatggactgaaccagatgattgtcatagaactgggcaccaatccgctgaagagctcaggaattgaaaatggggctttccagggaatgaagaagctctcctacatccgcattgctgataccaatatcaccagcattcctcaaggtcttcctccttcccttacggaattacatcttgatggcaacaaaatcagcagagttgatgcagctagcctgaaaggactgaataatttggctaagttgggattgagtttcaacagcatctctgctgttgacaatggctctctggccaacacgcctcatctgagggagcttcacttggacaacaacaagcttaccagagtacctggtgggctggcagagcataagtacatccaggttgtctaccttcataacaacaatatctctgtagttggatcaagtgacttctgcccacctggacacaacaccaaaaaggcttcttattcgggtgtgagtcttttcagcaacccggtccagtactgggagatacagccatccaccttcagatgtgtctacgtgcgctctgccattcaactcggaaactataagtccgggggtggcggatccgacttcgagccctccctaggcccagtgtgccccttccgctgtcaatgccatcttcgagtggtccagtgttctgatttgggtctggacaaagtgccaaaggatcttccccctgacacaactctgctagacctgcaaaacaacaaaataaccgaaatcaaagatggagactttaagaacctgaagaaccttcacgcattgattcttgtcaacaataaaattagcaaagttagtcctggagcatttacacctttggtgaagttggaacgactttatctgtccaagaatcagctgaaggaattgccagaaaaaatgcccaaaactcttcaggagctgcgtgcccatgagaatgagatcaccaaagtgcgaaaagttactttcaatggactgaaccagatgattgtcatagaactgggcaccaatccgctgaagagctcaggaattgaaaatggggctttccagggaatgaagaagctctcctacatccgcattgctgataccaatatcaccagcattcctcaaggtcttcctccttcccttacggaattacatcttgatggcaacaaaatcagcagagttgatgcagctagcctgaaaggactgaataatttggctaagttgggattgagtttcaacagcatctctgctgttgacaatggctctctggccaacacgcctcatctgagggagcttcacttggacaacaacaagcttaccagagtacctggtgggctggcagagcataagtacatccaggttgtctaccttcataacaacaatatctctgtagttggatcaagtgacttctgcccacctggacacaacaccaaaaaggcttcttattcgggtgtgagtcttttcagcaacccggtccagtactgggagatacagccatccaccttcagatgtgtctacgtgcgctctgccattcaactcggaaactataagtga

SEQ ID NO: 59 - protein, 1111 aa, Artificial Sequence
  synthetic
MMSFVSLLLVGILFHATQAEVQLLESGGGLVQPGGSLRLSCAASGFTFSSYIMMWVRQAPGKGLEWVSSIYPSGGITFYADTVKGRFTISRDNSKNTLYLQMNSLRAEDTAVYYCARIKLGTVTTVDYWGQGTLVTVSSASTKGPSVFPLAPSSKSTSGGTAALGCLVKDYFPEPVTVSWNSGALTSGVHTFPAVLQSSGLYSLSSVVTVPSSSLGTQTYICNVNHKPSNTKVDKKVEPKSCDKTHTCPPCPAPELLGGPSVFLFPPKPKDTLMISRTPEVTCVVVDVSHEDPEVKFNWYVDGVEVHNAKTKPREEQYNSTYRVVSVLTVLHQDWLNGKEYKCKVSNKALPAPIEKTISKAKGQPREPQVYTLPPSRDELTKNQVSLTCLVKGFYPSDIAVEWESNGQPENNYKTTPPVLDSDGSFFLYSKLTVDKSRWQQGNVFSCSVMHEALHNHYTQKSLSLSPGKSGGGGSDFEPSLGPVCPFRCQCHLRVVQCSDLGLDKVPKDLPPDTTLLDLQNNKITEIKDGDFKNLKNLHALILVNNKISKVSPGAFTPLVKLERLYLSKNQLKELPEKMPKTLQELRAHENEITKVRKVTFNGLNQMIVIELGTNPLKSSGIENGAFQGMKKLSYIRIADTNITSIPQGLPPSLTELHLDGNKISRVDAASLKGLNNLAKLGLSFNSISAVDNGSLANTPHLRELHLDNNKLTRVPGGLAEHKYIQVVYLHNNNISVVGSSDFCPPGHNTKKASYSGVSLFSNPVQYWEIQPSTFRCVYVRSAIQLGNYKSGGGGSDFEPSLGPVCPFRCQCHLRVVQCSDLGLDKVPKDLPPDTTLLDLQNNKITEIKDGDFKNLKNLHALILVNNKISKVSPGAFTPLVKLERLYLSKNQLKELPEKMPKTLQELRAHENEITKVRKVTFNGLNQMIVIELGTNPLKSSGIENGAFQGMKKLSYIRIADTNITSIPQGLPPSLTELHLDGNKISRVDAASLKGLNNLAKLGLSFNSISAVDNGSLANTPHLRELHLDNNKLTRVPGGLAEHKYIQVVYLHNNNISVVGSSDFCPPGHNTKKASYSGVSLFSNPVQYWEIQPSTFRCVYVRSAIQLGNYK

SEQ ID NO: 60 - DNA, 1746 bp, Artificial Sequence
  synthetic
atgatgtcctttgtctctctgctcctggttggcatcctattccatgccacccaggccgaggtacagcttttggagtcaggcggggggctcgtccaacctggggggtcactccggttgtcatgtgctgccagtggcttcacattctcatcttacattatgatgtgggttcgacaggcccctgggaaggggctggagtgggtttcctccatctacccctccgggggaattaccttctatgccgacacggtaaagggtcgcttcactataagtcgagataacagcaaaaatacgctgtatctccagatgaactctctcagggctgaggacacagctgtatattactgcgcgcggattaagttggggaccgtcacaacagtggattactggggtcaaggcactctggtaaccgtatcctcagcatccaccaagggcccaagtgtattcccgctggccccttcaagtaaatccacgtctggcggcacagccgctctcggttgcctggttaaggactacttcccagaacctgtcactgtcagttggaactcaggcgcattgacatctggtgtccatacattccccgcagtcctgcaaagctctggactttacagtcttagtagcgtagtgacagtcccatcttcaagtcttgggacccaaacttatatttgcaacgtaaatcataaaccctccaacactaaagtagacaaaaaagtagagccgaaatcttgcgacaaaacgcatacatgcccaccatgtcccgctccggaactcctgggcggcccgtccgtttttctctttcccccaaagcccaaggatacgcttatgatcagcagaacaccggaagttacttgtgtagtcgttgacgtgtctcacgaagatcccgaagtcaaatttaattggtatgtggatggcgtcgaagtgcacaacgcaaaaaccaaacccagagaggaacagtataacagcacgtatcgagtggtctccgtacttacggtcctccaccaggactggttgaatggcaaggagtacaagtgcaaagtgagcaataaagcgttgccagccccgatcgaaaaaaccatcagcaaggccaagggacagcctagagagccgcaggtttacaccttgccgccatcaagggatgaactgactaaaaaccaggtatccctgacctgcctggttaagggtttttaccccagtgatatagcggttgaatgggagtctaacgggcagccagagaacaactacaaaacgacacctcccgttctggattccgatggcagctttttcttgtattctaaactcaccgtggataaatcccgatggcagcaaggcaacgtcttctcctgcagcgtgatgcatgaagccttgcacaaccactatacccaaaagagtctcagcctgtcacccgggaaatccgggggtggcggatccctgcgtgcccatgagaatgagatcaccaaagtgcgaaaagttactttcaatggactgaaccagatgattgtcatagaactgggcaccaatccgctgaagagctcaggaattgaaaatggggctttccagggaatgaagaagctctcctacatccgcattgctgataccaatatcaccagcattcctcaaggtcttcctccttcccttacggaattacatcttgatggcaacaaaatcagcagagttgatgcagctagcctgaaaggactgaataatttggctaagttgggattgagtttcaacagcatctctgctgtttga

SEQ ID NO: 61 - protein, 581 aa, Artificial Sequence
  synthetic
MMSFVSLLLVGILFHATQAEVQLLESGGGLVQPGGSLRLSCAASGFTFSSYIMMWVRQAPGKGLEWVSSIYPSGGITFYADTVKGRFTISRDNSKNTLYLQMNSLRAEDTAVYYCARIKLGTVTTVDYWGQGTLVTVSSASTKGPSVFPLAPSSKSTSGGTAALGCLVKDYFPEPVTVSWNSGALTSGVHTFPAVLQSSGLYSLSSVVTVPSSSLGTQTYICNVNHKPSNTKVDKKVEPKSCDKTHTCPPCPAPELLGGPSVFLFPPKPKDTLMISRTPEVTCVVVDVSHEDPEVKFNWYVDGVEVHNAKTKPREEQYNSTYRVVSVLTVLHQDWLNGKEYKCKVSNKALPAPIEKTISKAKGQPREPQVYTLPPSRDELTKNQVSLTCLVKGFYPSDIAVEWESNGQPENNYKTTPPVLDSDGSFFLYSKLTVDKSRWQQGNVFSCSVMHEALHNHYTQKSLSLSPGKSGGGGSLRAHENEITKVRKVTFNGLNQMIVIELGTNPLKSSGIENGAFQGMKKLSYIRIADTNITSIPQGLPPSLTELHLDGNKISRVDAASLKGLNNLAKLGLSFNSISAV

SEQ ID NO: 62 - DNA, 2082 bp, Artificial Sequence
  synthetic
atgatgtcctttgtctctctgctcctggttggcatcctattccatgccacccaggccgaggtacagcttttggagtcaggcggggggctcgtccaacctggggggtcactccggttgtcatgtgctgccagtggcttcacattctcatcttacattatgatgtgggttcgacaggcccctgggaaggggctggagtgggtttcctccatctacccctccgggggaattaccttctatgccgacacggtaaagggtcgcttcactataagtcgagataacagcaaaaatacgctgtatctccagatgaactctctcagggctgaggacacagctgtatattactgcgcgcggattaagttggggaccgtcacaacagtggattactggggtcaaggcactctggtaaccgtatcctcagcatccaccaagggcccaagtgtattcccgctggccccttcaagtaaatccacgtctggcggcacagccgctctcggttgcctggttaaggactacttcccagaacctgtcactgtcagttggaactcaggcgcattgacatctggtgtccatacattccccgcagtcctgcaaagctctggactttacagtcttagtagcgtagtgacagtcccatcttcaagtcttgggacccaaacttatatttgcaacgtaaatcataaaccctccaacactaaagtagacaaaaaagtagagccgaaatcttgcgacaaaacgcatacatgcccaccatgtcccgctccggaactcctgggcggcccgtccgtttttctctttcccccaaagcccaaggatacgcttatgatcagcagaacaccggaagttacttgtgtagtcgttgacgtgtctcacgaagatcccgaagtcaaatttaattggtatgtggatggcgtcgaagtgcacaacgcaaaaaccaaacccagagaggaacagtataacagcacgtatcgagtggtctccgtacttacggtcctccaccaggactggttgaatggcaaggagtacaagtgcaaagtgagcaataaagcgttgccagccccgatcgaaaaaaccatcagcaaggccaagggacagcctagagagccgcaggtttacaccttgccgccatcaagggatgaactgactaaaaaccaggtatccctgacctgcctggttaagggtttttaccccagtgatatagcggttgaatgggagtctaacgggcagccagagaacaactacaaaacgacacctcccgttctggattccgatggcagctttttcttgtattctaaactcaccgtggataaatcccgatggcagcaaggcaacgtcttctcctgcagcgtgatgcatgaagccttgcacaaccactatacccaaaagagtctcagcctgtcacccgggaaatccgggggtggcggatccctgcgtgcccatgagaatgagatcaccaaagtgcgaaaagttactttcaatggactgaaccagatgattgtcatagaactgggcaccaatccgctgaagagctcaggaattgaaaatggggctttccagggaatgaagaagctctcctacatccgcattgctgataccaatatcaccagcattcctcaaggtcttcctccttcccttacggaattacatcttgatggcaacaaaatcagcagagttgatgcagctagcctgaaaggactgaataatttggctaagttgggattgagtttcaacagcatctctgctgtttccgggggtggcggatccctgcgtgcccatgagaatgagatcaccaaagtgcgaaaagttactttcaatggactgaaccagatgattgtcatagaactgggcaccaatccgctgaagagctcaggaattgaaaatggggctttccagggaatgaagaagctctcctacatccgcattgctgataccaatatcaccagcattcctcaaggtcttcctccttcccttacggaattacatcttgatggcaacaaaatcagcagagttgatgcagctagcctgaaaggactgaataatttggctaagttgggattgagtttcaacagcatctctgctgtttga

SEQ ID NO: 63 - protein, 693 aa, Artificial Sequence
  synthetic
MMSFVSLLLVGILFHATQAEVQLLESGGGLVQPGGSLRLSCAASGFTFSSYIMMWVRQAPGKGLEWVSSIYPSGGITFYADTVKGRFTISRDNSKNTLYLQMNSLRAEDTAVYYCARIKLGTVTTVDYWGQGTLVTVSSASTKGPSVFPLAPSSKSTSGGTAALGCLVKDYFPEPVTVSWNSGALTSGVHTFPAVLQSSGLYSLSSVVTVPSSSLGTQTYICNVNHKPSNTKVDKKVEPKSCDKTHTCPPCPAPELLGGPSVFLFPPKPKDTLMISRTPEVTCVVVDVSHEDPEVKFNWYVDGVEVHNAKTKPREEQYNSTYRVVSVLTVLHQDWLNGKEYKCKVSNKALPAPIEKTISKAKGQPREPQVYTLPPSRDELTKNQVSLTCLVKGFYPSDIAVEWESNGQPENNYKTTPPVLDSDGSFFLYSKLTVDKSRWQQGNVFSCSVMHEALHNHYTQKSLSLSPGKSGGGGSLRAHENEITKVRKVTFNGLNQMIVIELGTNPLKSSGIENGAFQGMKKLSYIRIADTNITSIPQGLPPSLTELHLDGNKISRVDAASLKGLNNLAKLGLSFNSISAVSGGGGSLRAHENEITKVRKVTFNGLNQMIVIELGTNPLKSSGIENGAFQGMKKLSYIRIADTNITSIPQGLPPSLTELHLDGNKISRVDAASLKGLNNLAKLGLSFNSISAV

SEQ ID NO: 64 - protein, 315 aa, Artificial Sequence
  synthetic
DFEPSLGPVCPFRCQCHLRVVQCSDLGLDKVPKDLPPDTTLLDLQNNKITEIKDGDFKNLKNLHALILVNNKISKVSPGAFTPLVKLERLYLSKNQLKELPEKMPKTLQELRAHENEITKVRKVTFNGLNQMIVIELGTNPLKSSGIENGAFQGMKKLSYIRIADTNITSIPQGLPPSLTELHLDGNKISRVDAASLKGLNNLAKLGLSFNSISAVDNGSLANTPHLRELHLDNNKLTRVPGGLAEHKYIQVVYLHNNNISVVGSSDFCPPGHNTKKASYSGVSLFSNPVQYWEIQPSTFRCVYVRSAIQLGNYK

SEQ ID NO: 65 - protein, 636 aa, Artificial Sequence
  synthetic
DFEPSLGPVCPFRCQCHLRVVQCSDLGLDKVPKDLPPDTTLLDLQNNKITEIKDGDFKNLKNLHALILVNNKISKVSPGAFTPLVKLERLYLSKNQLKELPEKMPKTLQELRAHENEITKVRKVTFNGLNQMIVIELGTNPLKSSGIENGAFQGMKKLSYIRIADTNITSIPQGLPPSLTELHLDGNKISRVDAASLKGLNNLAKLGLSFNSISAVDNGSLANTPHLRELHLDNNKLTRVPGGLAEHKYIQVVYLHNNNISVVGSSDFCPPGHNTKKASYSGVSLFSNPVQYWEIQPSTFRCVYVRSAIQLGNYKSGGGGSDFEPSLGPVCPFRCQCHLRVVQCSDLGLDKVPKDLPPDTTLLDLQNNKITEIKDGDFKNLKNLHALILVNNKISKVSPGAFTPLVKLERLYLSKNQLKELPEKMPKTLQELRAHENEITKVRKVTFNGLNQMIVIELGTNPLKSSGIENGAFQGMKKLSYIRIADTNITSIPQGLPPSLTELHLDGNKISRVDAASLKGLNNLAKLGLSFNSISAVDNGSLANTPHLRELHLDNNKLTRVPGGLAEHKYIQVVYLHNNNISVVGSSDFCPPGHNTKKASYSGVSLFSNPVQYWEIQPSTFRCVYVRSAIQLGNYK

SEQ ID NO: 66 - protein, 106 aa, Artificial Sequence
  synthetic
LRAHENEITKVRKVTFNGLNQMIVIELGTNPLKSSGIENGAFQGMKKLSYIRIADTNITSIPQGLPPSLTELHLDGNKISRVDAASLKGLNNLAKLGLSFNSISAV

SEQ ID NO: 67 - protein, 218 aa, Artificial Sequence
  synthetic
LRAHENEITKVRKVTFNGLNQMIVIELGTNPLKSSGIENGAFQGMKKLSYIRIADTNITSIPQGLPPSLTELHLDGNKISRVDAASLKGLNNLAKLGLSFNSISAVSGGGGSLRAHENEITKVRKVTFNGLNQMIVIELGTNPLKSSGIENGAFQGMKKLSYIRIADTNITSIPQGLPPSLTELHLDGNKISRVDAASLKGLNNLAKLGLSFNSISAV